European Patent Application EP 4 559 929 A1, published May 28, 2025. Title: USE OF β-1,3-GLUCAN SYNTHASE LIKE 5 IN IMPROVING CLUBROOT DISEASE RESISTANCE AND RELATED PRODUCT DEVELOPMENT IN CRUCIFEROUS CROPS. Applicant: Institute of Oil Crops Chinese Academy of Agricultural Sciences. Application US. The sequence listing filed with the application follows.

SEQUENCE LISTING (40 sequences)

SEQ ID NO: 1 - DNA, 8083 bp, Arabidopsis thaliana
  source 1..8083: mol_type = genomic DNA
ctgtcttaaatggacatttgtagtaacaaaaccgaccatcagcaaattaacgttaacgttgctctaatcgtgtgtatttttctaatgcttggtgaagcacatgcgaccatttgttgtgtcagaacaaaaggaagattccacatttagaatttagattataatcccacatgcctattatttaaacatatgtatactgtaataaattagtcccagaagagcatttcatcatactgtataattaatcaaatttaaaaaacatttgtgttgaagagaagatgactagattcacttgattttttttaatactgattggtcgtttgaccagtcaggatccagactgaaatattctcaaaaggtatgaactattttaatgaaatatttgagctgagaatttgcttatgggacattctatccttctaaagaaatcattagaaaatggagaaaaagttactagaaaaagagagggaaatggggcgagagtatgaagaaagggtcccatgtgaatctaataattgaaaagcaaatatgagatttattttagggttcttgttttagcgtccaaagcggtcgcagttgccgttcagcgacttttctctgtttatgaaataaaaacgctccacttgttcttttcttctttcaacccactttgttataactattaacaaatattgcttggtccaaattttattatactgaattattttagtttttttgtatcatcatcctcaatgttagttttgaaatcctaggtcagtaagtcaataacgaaaatgacaagtttaattttgtaattggaacttacatgtcacggtctttgtttacgatcattgccacgaattgtttagatacgggctttttttttctttccgtgttgatgattatcgtttcttcttacatatcttgatcaatcactaacatttacataacctacaattttgtaatataattgcaatactcgagatcttcaaatggtgatactgttaataaaattacgaacttttaatcatcatcaaaatctatagaaaaagatacataggaccaaaacaagcctaaaacaaagagttataatttacaaataaatgcatgtattttgttacttttgttaaggattttcatatcaatgcatgcataatgcattctctttttattttatttataatgcattcttttataatattcggatccaaaattatgaattaattccagattgccataaatgtctttctttgtttatgctgacttttttcttttcttaacttatatagtaagtaaaccagaaaggtggaagatacaaagcaatttcattgcattaataaacttcaaatgtattatccaataatcaaaatttatctagtaattcacaaaaaaaaaaaaatctgtctatcattcaaaatttcaccaatttggataaatatctagaaaattttaaaatacaattcaataacactattaacatatcaatcaatatataacattgcaaaagtttacttgatcattagtatattcattttaaggttaaaagatctttaagaaaaggaaattcaaattatattgttggaaaaaaatacaaatcaaagacagcaaaaaaagtaacaaaaaaaaaaggtagaagaaactgaaacgcggaaaggaggcaaaatcttctcgtcgtcgttgtcgccgtcttcagagctacaaacgaaaaaactcgcttccgtttcgatttctccattgttattgtttcttcagtgaagcttttttcttcgagaaatttctaagatctaccacatgctactatgagcctccgccaccgcaccgtcccgccgcaaaccggacggccgttggcggcggaagctgtcggaatcgaagaggagccgtacaatatcattcccgttaacaatctcctcgccgaccatccttcactccgttttcccgaggttcgtgccgccgctgctgctcttaaaaccgttggagaccttcgtcgtccgccgtatgttcaatggcgttctcactacgatctcctcgactggctcgccttgttcttcggtttccagaaagataacgttcgtaaccagcgtgagcatatggtgcttcatctcgcaaatgctcagatgcgtctctctccgccgccggataatattgattctctcgattccgcggttgttcgtcggtttcgtcggaaacttctcgctaactactctagctggtgttcgtatttggggaaaaaatcaaatatctggatctcagatcggaaccctgattcgagacgagagcttctctatgttggactctatcttctcatttggggagaggctgcgaatcttcggttcatgcctgaatgtatctgttacatcttccataacatggcctctgagctcaacaaaatcttagaggattgcctcgatgagaacaccggccaaccttacttgccttctctctcaggcgaaaacgctttcttaaccggcgtcgttaaacctatttacgatactatccaagctgagattgatgagagcaagaacggtacagttgcgcattgtaagtggaggaactacgacgatatcaatgagtacttctggactgatcggtgtttcagcaaattgaaatggccgcttgatttgggaagcaatttctttaagagtagaggcaaaagtgtagggaaaactggtttcgtggagcgcaggacgttcttctacctttacaggagttttgatcgactttgggtgatgctagctttgttccttcaagccgccattatagtagcttgggaggaaaagccagatacctcgtcggtaacaaggcagctgtggaatgctctgaaggcaagagatgttcaggtgagactattgaccgtgttcttgacatggagtggtatgcgactcttgcaggctgtgctggacgcggcttcacaatatcccctcgtttccagagagaccaaaaggcattttttcagaatgctgatgaaggttatagctgccgcagtttggattgtagctttcactgtcctctacactaacatctggaagcagaagaggcaagacaggcagtggtccaatgccgcgacgactaagatataccaattcctttacgctgtgggggccttcttggtgcccgaaatcctggctttggctttgtttattatcccatggatgagaaacttcctggaagagaccaattggaaaatattctttgctctaacttggtggtttcaaggcaaaagctttgtgggtcgaggtttgagagagggtttagtggacaacatcaagtactcgactttctggatctttgtcctagctacaaagtttacatttagttacttcctgcaggttaagccaatgattaaaccctcaaagctgctatggaacttaaaggatgtcgattatgagtggcatcagttttatggagacagcaataggttttctgtcgcattgttatggttgccagttgtgttgatatatctgatggatatccaaatttggtacgcaatctattcttcgattgttggtgctgttgttgggctgtttgatcatctgggggagatcagggacatgggacagctgaggctaaggtttcaattctttgctagtgctattcaattcaacctaatgcctgaggaacaactcctgaatgctagaggctttggtaacaagttcaaggacggcattcataggtagtccgtggaagcatgctactaatattcctaaataattttctgtacaacgcttgacttgactgtacaagctgtgaaattttacttttgttaacgcagatgctgcatataattaaatttttcaatattgtaataacttgaggttgtgtactgtatgcagattgaagctaaggtatggatttgggaggccgtttaagaaacttgagtcgaatcaggtcgaggccaacaagtttgcgttgatctggaacgaaatcatcttagctttcagagaagaggatatagtttctgatcgtgaagtagagctactggagctgccaaagaattcctgggatgtgacggttattcgctggccgtgtttcttgttgtgcaatgagcttttgcttgcactgagccaggccagagagctgatagacgcacctgataaatggctgtggcacaaaatatgcaagaatgaatacaggcgttgtgctgtagttgaggcatatgacagcatcaaacatctattgctctcaatcatcaaagttgacactgaagaacattcgataattacggtcttctttcagataattaatcagtccattcagtcagagcagttcaccaagacctttagagtggacctgctgccaaaaatttatgaaacactgcagaaattggttgggctggtaaatgatgaggaaacagatagtgggcgggtggtgaatgttctgcagtctctttatgagattgcaactcgacagttctttatagagaagaagacaactgaacagctatctaatgaaggtttaactcctcgagacccagcctcaaagttgctgtttcaaaatgctattaggcttcctgatgcaagcaatgaagacttctaccggcaggttaggcgtttacacacgattctcacctctagggactctatgcacagcgtccctgtgaatctagaggcgagacggcggattgctttcttcagtaattcgcttttcatgaacatgcctcatgcccctcaggttgagaaaatgatggcgttcagtgttctgactccatattacagtgaggaagttgtatacagcaaagaacagctccgaaatgagactgaggatgggatttccaccctatactacctgcagacaatttatgctgatgaatggaaaaatttcaaggaacggatgcatagggaaggaatcaagacagatagtgagttgtggacaaccaagctgagagacctcaggctttgggcttcctacagaggtcagacattggcacgtacagttcgtgggatgatgtactactaccgggctcttaagatgctcgcttttcttgactctgcgtctgaaatggacattcgggagggtgctcaggagcttggttcagtgaggaatttgcagggagaactgggtggtcaatctgatgggtttgtctctgaaaacgaccgatcttccttaagcagagcaagtagttccgtgagtacgctgtataaaggccatgagtatgggactgcattgatgaaattcacatatgttgtggcgtgtcagatctacgggtctcaaaaagcaaagaaagagcctcaggcagaggaaattctgtatctgatgaagcagaacgaagctctccgtattgcatatgtggatgaggtgcctgcgggaagaggagagactgattattactccgttctggtgaaatacgatcaccagttggagaaggaagtggaaatattccgtgtgaagctacctggtccagtgaagctgggcgagggaaagccagagaaccagaatcatgcaatgatctttacccgtggtgatgctgttcagaccattgatatgaaccaagacagttattttgaggaagctctcaagatgagaaatttgctccaggagtacaaccattatcatggtatcagaaaaccaactattcttggtgtcagggagcatatcttcacgggatcagtctcgtcactggcgtggttcatgtctgctcaggagacaagttttgtcactcttggtcagcgtgttcttgcaaacccactgaaggtcagaatgcattatggccaccctgatgtatttgacagattctggttcttgagtcgaggcggcatcagtaaggcttccagagttataaatatcagtgaggacatctttgccgggtttaactgcacgttaagggggggaaacgtcacccaccacgagtacattcaggttgggaagggtccacaatttggattatttctaactaactatactgctacaacgtttttttaacgtttttaacgtttattaattatgcaatctacttttgttataattatgtaatttaacgttttttaatcttctaaattcaaaaaatttgagtaacctttgtctttatgcatttttcaggtcgggaagggacgggatgttggattgaatcagatatcaatgtttgaggctaaggtagccagtgggaacggagagcaggttctcagccgagatgtgtaccggctcgggcacaggcttgatttcttcagaatgttatcatttttctacacaactgtagggtttttcttcaacacaatgatggtcattcttactgtttacgctttcctctggggacgggtttatctggctctcagcggggttgagaagtccgctctagcagacagtacggacaccaacgccgcgcttggggtgatcctgaaccagcagttcatcattcagctcggtctgttcactgccctgccaatgattgttgaatggtctctcgaggagggtttccttctagcgatatggaatttcattcgaatgcagattcagctttcagctgtcttctacacattctcaatggggaccagagctcactatttcggtcgaactattctccatggtggggccaagtatagagccactggacgtggatttgttgtcgagcacaagggattcactgagaactaccgactgtatgcacgcagtcactttgtgaaggccatcgagcttgggctgatcctcatagtctacgcttcgcacagtccgattgccaaagactcgttgatttacatagccatgactatcaccagctggtttcttgtgatttcatggataatggccccatttgtgtttaacccatcaggattcgactggcttaagacagtctatgactttgaagacttcatgaactggatctggtaccaaggcagaatctcaacgaaatctgaacaaagctgggaaaaatggtggtacgaggaacaggaccacctgagaaacaccgggaaggcaggattatttgtggagatcatcttggtcctccggtttttcttcttccagtatgggattgtataccagcttaaaattgcaaacggatccaccagcctttttgtctacttgttctcatggatatacatctttgctatatttgtgctcttcctagtcatccaatacgcccgtgacaagtactcggcaaaagctcacatacggtacaggcttgtccaattcctcctgatcgtgcttgctatactggtgattgttgctttgctcgagttcacgcatttcagcttcatcgatatcttcacaagccttcttgcattcatcccaactggctggggaattctgctgatcgcacagactcaaaggaagtggctgaagaattacactattttctggaatgctgttgtctctgttgctcgcatgtatgacatattgtttgggatactcataatggttccagtagcgttcttgtcatggatgcctggattccagtcaatgcaaacgaggatattattcaatgaagcttttagcagaggacttcgcatcatgcagattgtcactgggaagaaatcaaaaggcgatgtctaagtttaaaaaacggtaaagctccttgttctcaacaccttatgttatgatcgtttaaatcctggatttcacaccaatgcgggctttaaatttgtgtaggtcttaagaagtaaatggtagttcaaatcctattggtatgtggcgaaggaatcagttggaggttagttttcccgaaacaaccgaattcgaagttttgtttcgtctaaagaaaaactcagatgctgatgatttatctttgtattttaaacaggtttttggagagtttggttggatgaggaatcgggaagttggtttgattcggttagatgggtttagggagatatttgattgtcagtgtgtgtggagggaactctgattcttgtatggtttttgttctaaaggtacagcaatttgtgtagtgaggctttgtgtatttgttctccttctctcattatagagctttagagcatttttagtttatattcagattgttatctaatgtcatctcgcagagcttttgttcacatttcacatcttttcttctccttcttagtagagatcagtttcagattagatacttgtccatattccactactctcgtctattatcggtttctgcttgtcaatttctgggtccaaaattgaaata

SEQ ID NO: 2 - DNA, 10394 bp, Brassica napus
  source 1..10394: mol_type = genomic DNA
cttccttctttgccgtctctcttgaagctaagtacaccgatatggccgcctttaagtatgttaaatgcaaacacaaatcgattatgttcatctcataagttatgtgaatatttttagctagtaattgggtataacatgttttgtaggtattttgtgatcgcaaacgctgtcgtgagtgtttacagctttctagttctgtttcttcctaaggagagtttactgtggaagttcgtcgtcgtcttggatttggtaataattgttatttggtttagtacttctcttcgttcattaattcatttgcattctatctctaagcatagtttttttctaaaggtaatattattgttgatatctagtagtttgatgtgttcagaggaataaaagcatttttattggtgaaatactgaaaaataataaaatgttgattattatagttcaaataaacaattgttttctagaagaacataaagtaatcacaatattatattttgcatgagagttttttcacgaaattctcatatttcctcttattatcatttatcgttgagatactttctaagaactctttaatggagatgttctagtaaattaatctttgaacgaaaagttaaaacatacactttcaaaaaaaaaaagttaaaacaaataaacttgaatgtaatgtgtcttagtcacacgcttattataggttgttaggtgacgactatatcagcatacatacgaattgtcattaacttttgacatttttggtgaatgtattggaggtgatgacaatgctactaacgtcaagcatatcagcggcgttagcggtggcgcaagtgggaaagaaaggaaacgcaaacgcaggttggcttccaatttgcggccaagttccaaagttttgcgatcaggtcaccggagctctcattgccggcttcgtcgcactcgtcctctacgtcttgttactcttatactctcttcactccgtcgtcgatccttttcttctccagaaatcttgaatctaacttcttttttcactttcagtatcggttaatatacgttttaatatctatactataacgtcgtttgtgtattgtatttatatgttttctgttttaggtgtcgagattgtcatagtatttcatttttatggactaattaacattatagactgaaccacctctcataaactcttactcataattaaaaaaaaaaatcaatgcttcatatatacatctctgtcaatcattggattcgtatttattatagtatcaacaaatttgtgatacaaacctaaacatgtgcaatatctttagctaacgaaatggatatagatacatcttccctagctatggaaatgagtatttgatcaaaacgtaattgcacttgttagttagtcatttctctcagtgtaacaaaacaccatttatgaaaaaacactgagcatgggcaagtttcgtcttcacctccgttaatcttttgcatcgtaaaaacaatcgatgttacaaaacatgttttgttttaacgttgtaaaaatatcaggcttgatttgaatgtcatgttatgccgactttactagtttgtgtaaccaactaagctattaaaatatgcgtaattacaaaactgtcagatttagtttcacaaaatctttgtaacttcgcggtttttgatatggaagttgctacaaaaactgacttgtgatattataatctttcggcaagaaaaatatataatactaatttcagaaagtattctgttgaattgttgatcaccaaatacacataaaccggcagatgttgacatgtttacgtgggatcactgggatagaagttttgcttctgtattagtatcgcgaaccggtttgtagtagcgaaaataacattattattttcagatttcatcatcgtcaaattcaacgttacatttgaacaggcttgtaaaaagtggacatgtggcatgagtaaaagataaagaaaattgtgagcctttttgttaatacgaaaaagccgaaaacgttattatttctatcatcggcaaatttaatgttaaatttgctccacatcattcagagggtatatgtatatttttctaatgcttcggtgaagcacatgcgaccatttgttgcgtcagaagtcagaacaaaaggaagattccatctaatggattataatcccacatgcccatttttaaaactagacaaaataacttataatagtcccataagagcattaagacaaactgaaccaaaaagaatcttaaatgctggtgaatctagtctcgaatgctgctgaacactcctgatattagaatttggcagaaaatattcatactaataacagtaaatacatttcaaaacaagaaaatagtagtagtaaataaaaacaattaatatgttattattgtttctcttagctgttaccattacattaacaatttacattcaatccttttaatgaaaaatattataaaatattaaaagaagttattagaaaaggagagggatatgggggggggggggggagagcatggaggggtcccatgtgtgtttcgaaaagcagcaaacatgactttgtaaagtcttgttttagctagagttccaaaaaaaaaagagttcaaaaaaaaagaaaaaaaaaagtcttgttttagcgtccaaagcggtctcactcgccgttcagctgttaaattttcttgaaataaatcgctccacttgttttttatttttgtttctttcaacccacttgtattaataacaataatgatattgctaatcttgaacaaatcgtggattgtcttttcttccagtgatatcatccttagtcaaaacatctcaaattaaataaatatatagttgtgaattaaaaaaaaaggtatagagtttataaaattagcatttgcgaatgtttttaaaagtttggcgtttgtatagatcactgtcagtgtcatgaatcattcggtgacagcaaatttgtatatgccaaaaaagagagttgatacttgccattctcgatattttgaattttttttcgtcgacatacaaactcaacattttcgaaatcttagattaaaaacaaaatggacaaaacgatacttattaatgaattatgtactagcgtctaaacattagtaacatagatataattataagaacaagaaacatatatgcacaaagcctcaaaccaaatttaaatagtgttacgaaacaagggatgtacttgttatgaaaaattaatgtataaccattcttagcattttttacctaacccttaaactttataaagaaaaatatgtaacatttcggtgtgtggtatataaaagtattttgaaaatcgatttgattatttctattattaaaatgtacttactttttttatcacacatttatttacaatttcagagttaaacatgattaagacaaagtagtgaaaatatagatgatctaccagaaaatcatttgctttctgagtgagatcaaaataaaggcaaaaataatgtgatgattgtatattaaacaattattttgaatttgaaaagaataactcatcgaatgaagcctatgaaccgagtaagcggtgaagcggttggaccgtcacaaaaattatgaccaacaagaaaataaaattgatattagtgaatgatatattttggaaagtaataaattggttccagatttcaatacatcaatgtttttctaatgctgacttgcttttcctctttttcttacatgataaggaaacgagagaggtcgaagaaacaaagaaacttcctaagcatttagcaacgcatcttcaaaaaatctagtatttaccaagtaaaatcatacaaaataaggaaaaaaagaagaatatatttcccaatttggttttcacccgaaaaaaaaactgtcttaacaaaatcttaatgcaccaaatcatataagaactttatttgaccattgtcattagttttttccttatggtaatggatcttcaaataatttaaattaaattaaaaaaaaaagaaaagagaaacaaaaacgcggaaaggagagcccaaatcgtctccgtctgtcattgtcgcagtctctaaaagagaaaaacaaatcgcaacgcttctctctctctccctatcgtttgaatcagtctctcaagatccaccaccaccacacatgctactatgagcctccgccaccgcaccgtcccctctcaacccggacggcccccggcggcgggcgcaatcgaggacgagccctacaacatcatccccgtcaacaacctcctcgccgaccacccctccctccgctaccccgaggtccgcgccgccgccgccgccctcaaaaccgtcggcgacctccgccgccccacctacgtccaatggcgcccccactacgacctcctcgactggctcgccctcttcttcggcttccagaaggacaacgtccgcaaccagcgcgagcacctcgtcctccacctcgccaacgcccagatgcgcctcaccccgccgccggacaacatcgattccctcgatcccgccgtcgtccgccgcttccgccgcaagctcctcggtaactactccagctggtgctcctacctcgggaggaagtccaacatctggatctcggatcggagccccgattcgcggcgggagcttctctacgtcggcctctacctcctcgtctggggcgaggcggccaatcttaggtttatgcctgagtgtatctgttacatcttccacaatatggcctcggagcttaacaagatcttagaggattgcctcgacgagagcacggggcagccgtattctcctaagatcacgggggagaatagtttcctaaacggcgtcgttaagcctatctacgacacgatcagagctgagattaatgagagcaagaacgggacggagccgcattgtaagtggaggaactacgatgatattaatgagtacttctggacggataggtgttttagtaaattgaaatggccgattgatttggggagcagtttcttcaagaacagcagaggtagcggagttgggaagacaggttttgtggagaggaggacgtttttctacctctacaggagctttgataggctttgggtgatgcttgctttgtttcttcaagctgctattatagttgcttgggaggagaagccgggtggagggtcggtgacgagtcagctctggaatgcgttgaagtcgacggatgttcaggtgaggcttttgactgtgttcttgacgtggagtgggatgaggttgttgcaggctgtgttggacgctggctcgcaacggtctcttatttctagagagaccaaacggctgtttttcagaatgttgatgaaggttgtggctgctacggtttggatagtagcgtttattgttctctacacgaacatctggaagcagaggaagcaagataggcagtggtccagagccgcgaatgataagatctatcagttcctttacgctgtggtggctttcttggttcctgagatcctggctttggctctgtttatagtcccgtggataaggaactttctggaagagacgaattggaagatattctttgctttgacttggtggttccaggggaaaagctttgtgggtcgaggtttgagagaggggttggtggacaacatcaagtactcgactttctggatctttgtccttgcaacgaagttcacgttcagctacttcctgcaggttaagccaatgattaaaccctcgaagctgctatggaatttgaaggaggtggattatgagtggcatcagttctttggcgagagcaataggttttctgtcttgttattgtggctgccagtggtgttgatatacctgatggatatccaaatttggtacgcgatctattcttcgattgttggtgctgttgttgggctgtttgatcatctgggggagatcagggacatgggacagcttaggctgaggtttcagttctttgctagcgctattcagttcaacctaatgcctgaggaacaactcctgaatgctagaggatttggtaacaagcttaaggacgccattcataggtaagtctattgaagcatgttactgatatttctatataatttactatatagagtttgtctttaaagtacaagctatagtattttagttttgttaaagcagattctccgcaatgaactcgactttttcacattgtaataacattgagtttgtgtactttatgcagattgaagctgaggtatggattggggcggccgtttaagaaactcgagtccaatcaggttgaggctaacaagtttgcgctgatctggaatgagataatcttagctttcagagaggaggatatagtctctgatcgagaagtagagctgctggagctgccaaagaattcctggaatgtgacagttatccgctggccgtgtttcctgttgtgcaacgaacttttgcttgcactgagccaggcgaaagagctggttgacgcacctgataaatggctgtggcacaagatatgcaagaatgagtacaggcggtgtgctgtggttgaggcatatgaaagcatcaaacatctgttgctctcaatcatcaaaattgacactgaagaacataaaattgttacaattttctttcagatgattgaggtgtctattcagggtgagcagttcaccaagaccttcaaagtggaccttttgccaaagatttatgagacactgcagaagttggttgggctgttgaatgatgagaaagtggatgttgggcgagtggtgaatggtctgcagtctatttatgagattgcaacacgacagttcttcctagaaaagaagacgactgaacagctatctactgaggggttaactcctcatgatccagcctcaaagttactgtttcagaatgctgttaggcttcccgatgcaagcaatgaagacttcttccggcaggttaggcggttacacacaattctcacttctagggactctatgcacagcgtccctgtgaatctagaggcgagacggcggattgccttcttcagcaattcgctcttcatgaacttgcctcatgcacctcaggtggagaaaatgttggcgttcagtgttatgactccatactacagcgaggaagttgtatacagcaaagaacagctccgaaatgagactgaggatgggatttcaaccttgtattacctgcagacgatttatgccgacgaatggaaaaattttaaggaacggatgcgtagggaaggtataaagacagatgttgagttgtggacaaccaagctgagagagctcaggctttgggcttcctacagaggtcagactttggcacgtacaattcgaggaatgatgtactattacagggctcttaagatgcttgcttttcttgactctgcgtctgaaatggacattcgggaggatgctcaggagcttggttcaatgaggagttcgcagggaaatcgattggatggggtggacgatgtaaatgacggatcttctctaagcagagcaactagctctgtgagcatgctgtataaaggccatgagcatgggactgcattgatgaaattcacatatgtcgtggcgtgccagatctatgggtctcaaaaagcgaagaaggagcctcaggcagaggaaattctgtatcttatgaagcaaaacgaagccctccgtattgcatatgtggatgaggtgcatgcgggcagggaagagactgagtattactccgttctggtgaaatacgatcacacgttggagaaggaagtggagatattccgtgtgaagctacctggtccggtgaagctgggtgagggaaagccagagaaccagaatcatgcaatgatctttacccgcggtgatgctgttcagaccatagatatgaaccaggataattattttgaggaggctctcaaaatgagaaatttactccaggagtttaggcattatcatgggatcagaaaaccaactattcttggtgtcagagagcacatcttcacgggttctgtctcgtctctggcttggttcatgtctgctcaggaaacaagtttcgtcactctgggtcagcgtgttctagccaacccgctgaaggtcagaatgcattatggtcaccctgatgtatttgacagattctggttcttgagtcgaggtggcatcagcaaagcttctagagttataaatatcagtgaggacatcttcgccgggtttaattgcacattgcggggcggtaacgtcacccaccacgagtatattcaggtagggaaatgttcatcatttggatattctaactaattttatacatcgacaacaatactataattccactttttttgttataacctttttgtgtgtgcatatgtattcaggttgggaagggtcgagatgttggattgaatcaaatatcaatgtttgaggctaaggtagccagtgggaatggagagcaggttcttagccgagatgtgtacaggttgggtcataggctcgatttcttcagaatgttatcatttttctacacaacggtggggtttttcttcaacacgatgatggtcattctcactgtctacgctttcctctggggccgggtttatcttgctctgagcggtgttgagaagtccgctctagcagacagcacagacaccaacgcagcgcttgctgtgatattgaaccagcaattcatcattcagcttggtctcttcacagctctgccaatgattgtggaatggtctctcgaggagggtttccttctcgcgatatggaacttcattcggatgcagattcagctttcctctgtcttctacacattctcaatggggaccagagctcactattttggccgaaccattctccatggtggagcaaagtacagagccactgggcgtggatttgttgtcgagcacaagagcttcactgagaattaccgtctatacgcacgcagtcactttgtgaaggccatcgagcttgggctgatcctcatagtctacgctacgcacagtcccatcgccaaagactcattgatctatatagctatgactctcaccagctggttcctcgtgatatcatggatactggccccttttgtgttcaacccgtcaggattcgactggcttaagacggtctacgacttcgaaggcttcatgaactggatctggtatcaaggcaggatctcaacgaagtccgaacagagctgggagatatggtggtatgaggaacaggaccacctgagaaccaccggtataccaggaagaatcgtggagataatcttggaccttcggtttttcttcttccagtacgggattgtataccagctcaaaatcgcaaacggatcaaccagcattctcgtctacttactctcatggatatacatcttcgcagtgtttgtgttcttcctagtaatccaatacgcccgtgacaagtactctgcgagaaaccacatacggtacaggctcgttcagttcctcctgatcgtgtttggtacactggtgattgttgctctcctcgagttcacgcatttcagcttcgtggatatcttcacgagtcttcttgcgttcgtcccaaccggctgggggatcttgctgatcgcacaggcgttgaggcctgcgctgcagaagatcgggcttatctggaacgcggttatctcccttgctcggttatatgacatactgttcgggatagtcatcatggttcccgtagcgttcatgtcgtggatgcctgggtttcagtcgatgcaaacgaggatcttattcaatgaagcttttagcagagggcttcgtatcatgcagattgtcactgggaagaaatcaaaaggcgatgtcgaagttgaaaaaagaaggtaaagcttcttatttacccaaacatctttttatgttctgtttgtttggaatcttaaattacaacaacactaatgcaaagcttttacaacttgtgtaggtcttgaggtatatggtaatttaaaagttgctggtttgcggcgatgtgacctgttggaggttagttttgtattcttacaagttatgcttcttgtctgaataggaactcagacacccgtgttttgtcttcttcttattaaaccaggtttttggagagctttggttgaggaagctattcgattagataaatcttttagtgggggagacatatatatatacatttgtcagtactttgttagtgtgtggaagtggggacgactctgattctgattccttatgtggttattgtctgaaacgttacagcattttgtgaagtaggcttttgtgcaagatttgatctctttctctcattgtagagctttagagcattttttagtatatgtttaatctttgattttctaatgtcatttgcattcatattcacatcttcttcgttggtcttaaaccagttttcagatgcttatccattgtccacttctctatgtatctgtttcttctgtttgttttcagtattgtcttttattctttaatcagttttatttggacc

SEQ ID NO: 3 - DNA, 10431 bp, Brassica napus
  source 1..10431: mol_type = genomic DNA
agtgagtttgttctccagcgagccggagaaggcatcaacgcaaacctggaggaacagattgaccggtatgttcattaacgctgcaagccagctttgatgttagctgcgtaaagatccctgcgtttacatcaaaacattacattgtttgctgtgactaaggtaacagagtaaacgtgtaaaatactctggtgttttggagaaaacaaacttacatggagcccttaattgcatctatggcagcttgtgctgagaggaaaccttcaacgtccacttttccttgtaggttactaatatatgcatattttatttaaatcaatccaaatatatgggtaaaaaactttatttgaggatgtactatatatatgaatgcctaagagtataatgtacaaaggtgaaacttgccttgacattgaaggagtagaggactgtttgctccatggtagtcatgtaagtgtgaagaatagagagatgaagatcctccaaaaaagcaatagtcttaataagttgtcctggtcttcttcttgaaagtttcttgatcatggcatcaaactctagcagcttcacctccacatcagccaagcacgactcgttctcagctgtttcttcccggagccctcctcctcctcctatacgactcatgtgactctaggcattgtagaagttgctcaagctctcttacaaactctattccacctatgatcgacgcttgatctctctgttatatacatgcatattaaaaaatattttaaaataatgaatacaatcacgaaatgaagatgtatatgtgttatcatgatacccattgaacgtaggatccagacaaaagagacttgaggttacgaagatgctcgttcatttgcttcctattcctagcgaccgcaatatgtctcattcgttagttttctacttcttcgcttgtcttgcttgtttttgctcttcacctcctttgtcatatcattcttgttctcactatctccttcttctcctccagtaaaccgacttgttattgtcgttaacgtctaaggattcacctaaaaaatttggtgcctgaaagaaaataaaggtgaagaaataattattaagataatataggtcaattgacttggaatcaaaattttcaccctgcaagttgacatggtttcatactaatgtgatacattaagacatagtttatggttttaatgattgttacctgatccatcaggcattataccaaaaggacaggcacggaggaactattcagttagcccatgctcctgcacaaatttatcaatcaactcatatctagaaggatatatgagaaaagaagtttctggtgttattaggagttgtgaggatgatgtttattaagaaataaactatataagcctttacatataaattacaaaataccttgattctcatccaagattccggtgtggatcgatttatcaatgacatatttgcaaaaaaaaataatagggttacctggaagatgggtgttggtgtttgctagaccaagcaactcatctttgcagaacctgaaacgttcttgaggaattggtgaacctgggtcagttaagtctttcaaacccgtctcaatattgaaccggatcgacacaggagagtcggacagcttgaagtccggacagctcaaagccgctaacagagtacacttaaccaacagtgaaaagatgtctgaatgtgtttaagcggtagacgttcacggtggcttaggtgagagtggcctgcaaagcatgaaaaattggaaacataaacaaatgaaataaatattgcaatcattaaaaataaactaaagcgcttgttaactttttcataatcaaaagacataagcatatggatgtctctacacggactatttgaattttaggtatgaataaaatatacgaaaaaagtaaaaaagaatcaacaatcacaacaatgatcatatcccaaatatttgaagataacaaaaacttatggagaataacgaagacatgaatgtattgatctccggtgaagaactattaggtttgaaagtttcataaccaaaacacaacaacgcgagaaaggattaaaaaacaaaacaaaactacatagtcaagccggatttaccttggcgtccatgaagagaatgttgaccctctctgtcgcgcttaacattcctatcttcccagaacctaagcaaacggacctgggcggtggaggtgcagcggctagctttcaaatcggcgagaaagacggaggaattagccattatcgactttgatttcttagaaaacagtttatgggaatgtagtaggattgtgagaatgatgtttctgggaagagcacatacctttttgtaggaggagcttcaccgcttgtaagagagatgagagtattgagtgagaaatcgttgagcttcatcgtggaggatggatttaaaaagggctttaagagtaagaatctgtaacaggtagattgctggatccgtaggaagaagatgaagcatctcgatcaaaaccctagggtatgatattgcaacggcggagaagagaatgagatgaaaccatagaattaaaaactctgcgtttcaggcatacgtcttactctgctttttaaagattgggctttataaaccaaaacaataacaaagaatgtagcccaaacggaaacagaataaatgaaacgcggtaaagtgaacagatgtcacataatgattggctgatttaattgtcctacgtggacagcttctctgatgctcatataacccttttagtataggttagatgatatcatccttagtcaaaagtcaaaacatctcaaattaaataagtatagagttgtgaatttttaaaaaagtatagagtatataaaattagcatttgcgaatgtttttaaaagtttggcgtttgtatggatcactgtcagtgtcatgaatcattcggtgactgcaaaattttatatgacaaaaaaaaaagagagttgatacttaccattctcgatattttgaaatttttttcgtcgttaatacaaactcaacattttcgaaatcttggattaaaaaaaaaaaatatggacaaaacggtacttattaattaattatgtactagcgtcttgacattattaatatagatataattataagaacaagaaacgtatatgcacaaaccctcaaaccaaatttaaatagtgttaaaaaacaagggatgtacttgttatgaaaaattaatatataaccattcttaacatttttacctaacccttaaactttataaataaaaatacgtaatatcccgatagaaatattttaaaattttgatttgattatttatgttatcaaagtgcatttatttttttttgtcacgtatatatttaaaatttcaacattaaaagtgtgtaagatggagtagtgaaaatatagacgacttaccataaaattatttgtgatatcatttgaataagactaaaacacggacaaaaataatatagtgattgcattgttattaaacaattatttggatttgaaaagaaataactcattgaatgaagcctatgagccgagtaaacggacgtggatagcttaagcggttggaccgtacaaaatttatgaccaacaagaaaatgaaattgattttttttttgacgaaaaaatgaaattgattttagaaagtaacaaaatggttccagatttcaatacttcaacgtttttttatgccgactttcttttcctcttttacttacatgataaggaaacgagagaggttgaagaaacaaagaaacttcctaagcatttagaaatgtatcttcaaaaaatctagtatttaccaagtaaaatcattcaaaataaggaaaaaaagaagaatctatttcccaatttggttttcaccgaaaaaaaaattgtcttaataaaatcttaatgcaccaaatcatataagaactttatatgaccattgtcattagttttttctttatggtaatggatcttcaaataatttaaattaaattaaaaaaaaaaaagagaaacaaaaacgcggaaaggagagcccaaatcgtctccgtctgtcattgtcgcagtctctcacagctaaataaaagagaaaaacaaatcgcaacgcttcaatatctctctcccaatcgtttgaatcagtcttcctcatcacaatcccccaaagatccaccacacatgctactatgagcctccgccaccgcaccgtcccctctcaacccggacggcccccggcggcgggcgcaatcgacgacgagccctacaacatcatccccgtcaacaacctcctcgccgaccacccctccctccgctaccccgaggtccgcgccgccgccgccgccctcaaaaccgtcggagacctccgccgccccacctacgtccaatggcgcccccactacgacctcctcgactggctcgccctcttcttcggcttccagaaggacaacgtccgcaaccagcgcgagcacctcgtcctccacctcgccaacgcccagatgcgcctcacgccgccgccggataacatcgattccctcgatcccgccgtcgtccgccgtttccgccgcaagctcctcggtaactactcgagctggtgctcgtacctcgggaggaagtcgaacatctggatctcggatcggaaccccgattcgaggcgggagcttctctacgtcggcctctacctcctcgtgtggggggaggcggcgaatcttaggtttatgccggagtgtgtctgttacatcttccacaatatggcctcggagcttaacaagatcctcgaggattgcctcgacgagagcacggggcagccgtactctcctagaatcacgggggagaatagtttcctaaacggcgtcgttaaacctatttacgagacgatcaaagctgagattaacgagagcaagaacgggacggagccgcattgtaagtggaggaactatgatgatattaatgaatacttttggacggataggtgttttagtaaattgaaatggccgattgatttggggagcagtttcttcaagagtagtagagggagaggcgttgggaagacaggttttgtggagaggaggacgttcttttacctctacaggagctttgataggctttgggtgatgcttgctttgtttcttcaagctgctattatagtcgcttgggaggagaagccgggtggagggtcggtgaggagtcagctctggaatgcgttgaagtcgagggatgttcgggtgaggcttttgactgtgttcttgacgtggagtgggatgagattactgcaggctgtgctggacgctgcctcgcaacggccgcttatttctagagagaccaagcggctgtttttcagaatgttgatgaaggttgtagctgctacggtttggataattgcttttattgttctctacacgaacatctggaagcagaggaagcaagacaggcagtggtccagagccgcgaatgacaagatctatcagttcctttacgctgtggtggctttcttggtccctgagatcctggctttggctctgtttatagtcccgtggataaggaactttctggaagagaccaattggaagatattctttgctttgacttggtggttccagggtaaaagctttgtgggtcgaggtttgagagaggggttggtggacaacatcaagtactcgactttctggatctttgtcctagcaacgaagttcacgttcagctacttccttcaggttaagccaatgattaaaccctcgaagctgctatggaatttgaaggaggtggattatgagtggcatcagttctttggcaagagcaataggttttctgtcttgttattgtggctgccagtggtgttgatatacctgatggatatccaaatttggtacgcgatctattcttcgattgttggtgctgttgttgggctgtttgatcatctgggggagatcagggacatgggacagcttaggctgaggtttcagttctttgctagcgctattcagttcaacctaatgcctgaggaacaactcctgaatgctagaggatttggtaacaagcttaaggacgccattcataggtaagtctattgaagcatgttactgatattcctttataatttactgtacagagtttgtctttacggtacaagttatggaattttagttttgttaaagcagattctcttaactcggcttttcaacattgtaataaccttgagtttgtgtactttatgcagattgaagctgaggtatggacttgggcggccatttaagaaactcgagtctaatcaggttgaggctaacaagtttgcgctgatctggaatgagataatcttagctttcagagaagaggatatagtctctgatcgagaagtagagctactggagctgccaaaaaattcctggaatgtgacagttatccgctggccgtgtttcctgttgtgcaacgagcttttgcttgcactgagccaggcgaaagagctggttgacgcacctgataaatggctgtggcacaagatatgcaagaacgagtacaggcggtgtgctgtggttgaggcatatgaaagcatcaaacatctgttgctctcaatcatcaaaattgacaccgaagaacataaaattattacaattttctttcagatgattgaggtgtctattcagggtgagcagttcaccaagaccttcaaagtggacctattgccaaagatttatgagacgctacagaagttggttgggctgttgaatgatgagaaagtggatgttgggcgagtggtgaatggtctgcagtctatttatgagattgcaacacgacagttcttcatagaaaagaagacgactgaacagctatctaccgaggggttaactcctcatgatccagcctcaaagttactgtttcagaatgctgttaggcttcccgatgcaagcaatgaagacttcttccggcaggttaggcggttacacacaattctcacttctagggactctatgcacagcgtccctgtgaatctagaggcgagacggcggattgccttcttcagcaattcgctcttcatgaacttgcctcatgcacctcaggtggagaaaatgttggcgttcagtgttatgactccatactacagcgaggaagttgtatacagtaaagaacagctccgaaatgagactgaggatgggatttcaaccttgtattacctgcagacgatttatgccgacgaatggaaaaattttaaggaacggatgcgtagggaaggtataaagacagatgttgagttgtggacaaccaagctgagagagctcaggctttgggcttcctacagaggtcagactttggcacgtacagttcgaggaatgatgtactattacagggctcttaagatgcttgcttttctcgactctgcgtctgaaatggacattcgggaggatgctcaggagcttggttcaatgaggagttcgcagggaaatcgattggatggtgttgacgatgtaaatgaccgatcttctctaagcagagcaactagctctgtgagcatgctgtataaaggccatgagcatgggactgcattgatgaaattcacatatgtcgtggcgtgccaaatctatgggtctcaaaaagcgaagaaagagcctcaggcagaggaaattctgtatcttatgaagcaaaacgaagcccttcgtattgcatatgtggatgaggtacatgcgggcaggggagagactgagtattactccgttctggtgaaatacgatcacacgttggagagggaagtggagatattccgtgtgaagctacctggtccggtgaagctgggtgagggaaagccagagaaccagaatcatgcaatgatctttacccgtggtgatgctgttcagaccatagatatgaaccaggataattattttgaggaggctctcaagatgagaaatttgctccaggagtttaggcattatcatgggatcagaaaaccaactattcttggtgtcagagagcacatcttcacgggttctgtctcgtctctggcttggttcatgtctgctcaggagacaagtttcgtcactcttggtcagcgtgttctagccaacccgctgaaggtcagaatgcattatggtcaccctgatgtatttgacagattctggttcttgagtcgaggtggcatcagcaaagcttctagagttataaatatcagtgaggacatcttcgccgggtttaattgcacattgcggggcggtaacgtcacccaccacgagtatattcaggtagggaaatgttcatcgtttggatattctaactaatttatacatcgacaacaatactataattccacttttttgttataacctttttgtgtgtgcatatgtattcaggttgggaagggtcgagatgttggattgaatcaaatatcaatgtttgaggctaaggtagccagtgggaatggagagcaggttcttagccgagatgtgtacaggttgggtcataggctcgatttcttcagaatgttatcatttttctacacaacggtggggtttttcttcaacacgatgatggtcattctcactgtctacgctttcctctggggccgggtttatcttgctctgagcggtgttgagaagtccgctctagcagacagcacagacaccaacgcagcgcttgctgtgatattgaaccagcagttcatcattcagcttggtctcttcacagctctgccaatgattgtggaatggtctctcgaggagggtttccttctcgcgatatggaacttcattcggatgcagattcagctttcttctgtcttctacacattctcaatggggaccagagctcactattttggccgaaccattctccacggtggagcaaagtacagagccactggacgtggatttgttgtcgagcacaagagtttcactgaaaactaccgtctatacgcgcgcagtcactttgtgaaggccatcgagcttgggctgatcctcatagtctacgctacgcacagtcccatcgccaaagactcattgatctatatagccatgactctcaccagctggttcctcgtgatttcatggatactagccccttttgtgttcaacccgtcaggtttcgactggcttaagacggtctacgacttcgaaggcttcatgaactggatctggtatcaaggcagaatctcaacgaagtccgaacagagctgggagatatggtggtatgaggaacaggaccacctgagaaccaccggtctaccaggaagaatcatggagataatcttggaccttcggtttttcttcttccagtacgggattgtataccagctcaaaatcgcaaacggatcaaccagcattctcgtctacttactctcatggatatacatcttcgcagtgtttgtgttcttcctggtaatccaatacgcccgtgacaagtactcagcgagaaaccacatacggtacaggctcgttcaattcctcctgatcgtgtttggtacactggtgattgttgctctcctggagttcacgcatttcagcttcgtggatatcttcacgagtcttcttgcgttcgtcccaaccggctggggaatcttgctgatcgcacaggctttgaggcctgcgctgcagaagatcgggcttatctggaacgcggttatctcccttgctcggttatatgacatactgttcgggatagtcatcatggtccccgtagcgttcatgtcgtggatgcctgggtttcagtcgatgcaaacgaggatcttattcaatgaagcttttagcagagggcttcgtatcatgcagattgtcactgggaagaaatctaaaggcgatgtcgaagttgaaaaaagaaggtaaagcttttataacttgtgttctgtttatgtttgtttggaatcttaaattacaacaacaccaatgcaaagcttttataacttgtttaggtcttaaggtatatggtaacttaaaagtcgttggttttgcggcgatgtgatcagttggaggttagttttctcaagacatggaagttttataagttattgcttcttgtgtgaagaagaagtcatatacatccatgttttgttttgtcttcttcttaaagcaggtttttggagagctttggttgaggaatccggaagttagataatcttttagtgggggagacatatatatacacatttgtcagtactttgttagagtgtgtggaagtggggacgactctgattctggttccttatgtggttattgtctgaaacgttacagcattttgtgaagtaggcttttgtgcaagatttgatctctttctctcattgtagagctttagagcattttttagtatatgtttaatcttttgattttctaatgtcatttgcattcatatttcacatcttcttcgttggtcttaaaccagttttcagatgcttatccattgtccacttttctatgtatctgtttcttctgtttgttttcagtattgtcttttattctttaatcagttttatttggaccacaacacca

SEQ ID NO: 4 - DNA, 9344 bp, Brassica rapa
  source 1..9344: mol_type = genomic DNA
aaagtaataaaatggttccaaatttcaatacatcaatggttttctaatgctgacttgcttttcctcttttacttaaacgataaggaaacgagagaggttgaagaaacaaagaaacttcctaagcatttacaaatatatcttcaaaaaatctagtatttaccaagtaaaatcatacaaaataagaaaaaaaaagaagaatctatttcccaatttggttttcaccggaaaaaaaaaactgtcttaacaaaatcttaatgcaccaaatcatataagaactttatttgaccattgtcattagtttttttccttatggtaatggatcttcaaataatttaaattaaattaaaaaaaaagaaaaaagaaacaaaaacgcggaaaggagagcccaaatcgtctccgtctgtcattgtcgcagtctctaaaagagaaaaacaaatcgcaacgcttcaatatctctctctctctccctatcgtttgaatcagtctcccaagatccaccaccacacatgctactatgagcctccgccaccgcaccgtcccctcacaacccggacggcccccggcggcgggcgcaatcgacgaggagccctacaacatcatccccgtcaacaacctcctcgccgaccacccctccctccgctaccccgaggtccgcgccgccgccgccgccctcaaaaccgtcggcgacctccgccgccccacctacgtccaatggcgcccccactacgacctcctcgactggctcgccctcttcttcggcttccagaaggacaacgtccgcaaccagcgcgagcacctcgtcctccacctcgccaacgcccagatgcgcctctccccgccgccggacaacatcgattccctcgatcccgccgtcgtccgccgcttccgccgcaagctcctcggtaactactccagctggtgctcctacctcgggaggaagtccaacatctggatctcggatcggacccccgattcgcggcgggagcttctctacgtcggcctctacctcctcgtgtggggcgaggcggcgaatcttaggtttatgcctgagtgtatctgttacatcttccacaatatggcctcggagcttaacaagatcttagaggattgcctcgacgagagcacggggcagccgtattctcctaagatcacgggggagaatagtttcctaaacggcgtcgttaagtcagaacaaaaggaagattccatctaatggattataatcccacatgcccatttttaaaactagacaaaataacttataatagtcccataagagcattaagacaaactgaaccaaaaagaatcttaaatgctggtgaatctagtctcgaatgctgctgaacactcctgatattagaatttggcagaaaatattcatactaataacagtaaatacatttcaaaacaagaaaatagtagtagtaaataaaaacaattaatatgttattattgtttctcttagctgttaccattacattaacaatttacattcaatccttttaatgaaaaatattataaaatattaaaagaagttattagaaaaggagagggatatggggggggggagagcatggaggggtcccatgtgtgtttcgaaaagcagcaaacatgactttgtaaagtcttgttttagctagagttccaaaaaaaaaagagttcaaaaaaaaagaaaaaaaaaagtcttgttttagcgtccaaagcggtctcactcgccgttcagctgttaaattttcttgaaataaatcgctccacttgttttttatttttgtttctttcaacccacttgtattaataacaataatgatattgctaatcttgaacaaatcgtggattgtcttttcttccagtgatatcatccttagtcaaaacatctcaaattaaataaatatatagttgtgaattaaaaaaaaaggtatagagtttataaaattagcatttgcgaatgtttttaaaagtttggcgtttgtatagatcactgtcagtgtcatgaatcattcggtgacagcaaatttgtatatgccaaaaaagagagttgatacttgccattctcgatattttgaattttttttcgtcgacatacaaactcaacattttcgaaatcttagattaaaaacaaaatggacaaaacgatacttattaatgaattatgtactagcgtctaaacattagtaacatagatataattataagaacaagaaacatatatgcacaaagcctcaaaccaaatttaaatagtgttacgaaacaagggatgtacttgttatgaaaaattaatgtataaccattcttagcattttttacctaacccttaaactttataaagaaaaatatgtaacatttcggtgtgtggtatataaaagtattttgaaaatcgatttgattatttctattattaaaatgtacttactttttttatcacacatttatttacaatttcagagttaaacatgattaagacaaagtagtgaaaatatagatgatctaccagaaaatcatttgctttctgagtgagatcaaaataaaggcaaaaataatgtgatgattgtatattaaacaattattttgaatttgaaaagaataactcatcgaatgaagcctatgaaccgagtaagcggtgaagcggttggaccgtcacaaaaattatgaccaacaagaaaataaaattgatattagtgaatgatatattttggaaagtaataaattggttccagatttcaatacatcaatgtttttctaatgctgacttgcttttcctctttttcttacatgataaggaaacgagagaggtcgaagaaacaaagaaacttcctaagcatttagcaacgcatcttcaaaaaatctagtatttaccaagtaaaatcatacaaaataaggaaaaaaagaagaatatatttcccaatttggttttcaccggaaaaaaaaaactgtcttaacaaaatcttaatgcaccaaatcatataagaactttatttgaccattgtcattagttttttccttatggtaatggatcttcaaacaatttaaattaaattaaaaaaaaaaagaaaagagaaacaaaaacgcggaaaggagagcccaaatcgtctccgtctgtcattgtcgcagtctctaaaagagaaaaacaaatcgcaacgcttcaatatctctctctctctctctccctatcgtttgaatcagtctctcaagatccaccaccacacatgctactatgagcctccgccaccgcaccgtcccctctcaacccggacggcccccggcggcgggcgcaatcgaggacgagccctacaacatcatccccgtcaacaacctcctcgccgaccacccctccctccgctaccccgaggtccgcgccgccgccgccgccctcaaaaccgtcggcgacctccgccgccccacctacgtccaatggcgcccccactacgacctcctcgactggctcgccctcttcttcggcttccagaaggacaacgtccgcaaccagcgcgagcacctcgtcctccacctcgccaacgcccagatgcgcctctccccgccgccggacaacatcgattccctcgatcccgccgtcgtccgccgcttccgccgcaagctcctcggtaactactccagctggtgctcctacctcgggaggaagtccaacatctggatctcggatcggacccccgattcgcggcgggagcttctctacgtcggcctctacctcctcgtgtggggcgaggcggcgaatcttaggtttatgcctgagtgtatctgttacatcttccacaatatggcctcggagcttaacaagatcttagaggattgcctcgacgagagcacggggcagccgtattctcctaagatcacgggggagaatagtttcctaaacggcgtcgttaagcctatctacgacacgatcagagctgagattaatgagagcaagaacgggacggagccgcattgtaagtggaggaactacgatgatattaatgagtacttctggacggataggtgttttagtaaattgaaatggccgattgatttggggagcagtttcttcaagaacagcagaggtagcggagttgggaagacaggttttgtggagaggaggacgtttttctacctctacaggagctttgataggctttgggtgatgcttgctttgtttcttcaagctgctattatagttgcttgggaggagaagccgggtggagggtcggtgacgagtcagctctggaatgcgttgaagtcgacggatgttcaggtgaggcttttgactgttttcttgacgtggagtgggatgaggttgttgcaggctgtgctggacgctggctcgcaacggtcgcttatttctagagagaccaaacggctgtttttcagaatgttgatgaaggttgtggctgctacggtttggataatagcgtttattgttctctacacgaacatctggaagcagaggaagcaagataggcagtggtccagagccgcgaatgataagatctatcagttcctttacgctgtggtggctttcttggtccctgagatcctggctttggctctgtttatagtcccgtggataaggaactttctggaagagaccaattggaagatattctttgctttgacttggtggttccaggggaaaagctttgtgggtcgaggtttgagagaggggttggtggacaacatcaagtactcgactttctggatctttgtcctcgcaacgaagttcacgttcagctacttccttcaggttaagccaatgattaaaccctcgaagctgctatggaatttgaaggaggtggattatgagtggcatcagttctttggcgagagcaataggttttctgtcttgttattgtggctgccagtggtgttgatatacctgatggatatccaaatttggtacgcgatctattcttcgattgtcggtgctgttgttgggctgtttgatcatctgggggagatcagggacatgggacagcttaggctgaggttccagttctttgctagcgctattcagttcaacctaatgcctgaggaacaactcctgaatgctagaggatttggtaacaagcttaaggacgccattcataggtaagtctattgaagcatgttactgatattcctcctatataatttactatacagagtttgtctttacagtacaagctataggattttagttttgttaaagcagattctccgcaatgaactagactttttcacattgtaataacattgagtttgtgtactttatgcagattgaagctgaggtatggattggggcggccgtttaagaaactcgagtccaatcaggttgaggctaacaagtttgcgctgatctggaatgagataatcttagctttcagagaggaggatatagtctctgatcgagaagtagagctgctggagctgccaaagaattcctggaatgtaacagttatccgctggccgtgtttcctgttgtgcaatgagcttttgcttgcactgagccaggcgaaagagctggttgacgcacctgataaatggctgtggcacaagatatgcaagaatgagtacaggcggtgtgctgtggttgaggcatatgaaagcatcaaacatctgttgctttcaatcatcaaaattgacactgaagaacataaaattgttacaattttctttcagatgattgaggtctctattcagggtgagcagttcaccaagaccttcaaagtggaccttttgccaaagatttatgagacactacagaagttggttggtctgttgaatgatgagaaagtggatgttgggcgagtggtgaatggtctgcaatctatttatgagattgcaacacgacagttcttcatagaaaagaagacgactgaacagctatctactgaggggttaactcctcatgatccagcctcaaagttactgtttcagaatgctgttaggcttcccgatgcaagcaatgaagacttcttccggcaggttaggcggttacacacaattctcacttctagggactctatgcacagcgtccctgtgaatctagaggcgagacggcggattgccttcttcagcaattcgctcttcatgaacttgcctcatgcacctcaggtggagaaaatgttggcgttcagtgttatgactccatactacagcgaggaagttgtatacagcaaagaacagctccgaaatgagactgaggatggaatttcaaccttgtattacctgcagacgatttatgccgacgaatggaaaaattttaaggaacggatgcgtagggaaggtataaagacagatgttgagttgtggacaaccaagctgagagagctcaggctttgggcttcctacagaggtcagactttggcacgtacagttcgaggaatgatgtactattacagggctcttaagatgcttgcttttcttgactctgcgtctgaaatggacattcgggaggatgctcaggagcttggttcaatgaggagttcgcagggaaatcgattggatggggttgacgatgtaaatgacggatcttctctaagcagagcaactagctctgtgagcatgctgtataaaggccatgagcatgggactgcattgatgaaattcacatatgtcgtggcgtgccagatctatgggtctcaaaaagcgaagaaggagcctcaggcagaggaaattctgtatcttatgaagcaaaacgaagccctccgtattgcatatgtggatgaggtacatgcgggcaggggagagactgagtattactccgttctggtgaaatacgatcatacgttggagagggaagtggagatattccgtgtgaagctacctggtccggtgaagctgggtgagggaaagccagagaaccagaatcatgcaatgatctttacccgtggtgatgctgttcagaccatagatatgaaccaggataattattttgaggaggctctcaagatgagaaatttgctccaggagtttaggcattatcatgggatcagaaaaccaactattcttggtgtccgggagcacatcttcacgggatctgtctcgtctctggcatggttcatgtctgctcaggagactagtttcgtcactcttggtcagcgtgttctcgccaatccgctgaaggtcagaatgcattatggtcatcctgatgtttttgacagattctggttcttgagtcgaggtggcatcagcaaagcttctagagttataaatatcagtgaggacatcttcgccgggtttaattgcacattgcggggcggtaacgtcacccaccacgagtatattcaggtagggaaatgttcatcatttggatattctaactaatttatacatcgacaacaatactataattccactttttttgttataaccttcgtgtgtgtgcatatgtattcaggttgggaagggtcgagatgttggattgaatcaaatatcaatgtttgaggctaaggtagccagtgggaatggagagcaggttcttagccgagatgtgtacaggctgggtcataggctcgatttcttcagaatgttatcatttttctacacaacggtggggtttttcttcaacacgatgatggtcattctcactgtctacgctttcctctggggtcgggtttatcttgctctgagcggtgttgagaagtccgctctagcagacagcacagacaccaacgcagcgcttgctgtgatattgaaccagcaattcatcattcagcttggtctcttcacagctctgccaatgattgtggaatggtctctcgaggagggtttccttctagcgatatggaatttcattcggatgcagattcagctttcatctgtcttctacacattctcaatggggaccagagctcactattttggccgaaccattctccatggtggagcaaagtacagagccactgggcgtggatttgttgtcgagcacaagagcttcactgagaattaccgtctatacgcacgcagtcactttgtgaaggccatcgagcttgggctgatcctcatagtctacgctacgcacagtcccatcgccaaagactcattgatctatatagctatgactctcaccagctggttcctcgtgatttcatggatactggccccttttgtgttcaacccgtcaggattcgactggcttaagacggtctatgacttcgaaggcttcatgaactggatctggtatcaaggcagaatctcaacgaagtccgaacagagctgggagatatggtggtatgaggaacaggaccacctgagaaccaccggtataccaggaagaatcgtggagataatcttggaccttcggtttttcttcttccagtacgggattgtataccagctcaaaatcgcaaacggatcaaccagcattctcgtctacttactctcatggatatacatcttcgcagtgtttgtgttcttcctagtaatccaatacgcccgtgacaagtactcagcgagaaaccacatacggtacaggctcgtccagttcctcctgatcgtgtttggtacactggtgattgttgctctcctcgagttcacgcatttcagcttcgtggatatcttcacgagtcttcttgcgttcgtcccaaccggctggggaatcttgctgatcgcacaggctttgaggcctgcgctgcagaagatcgggcttatctggaacgcggttgtctcccttgctcggttgtatgacatactgttcgggatagtcatcatggttcccgtagcgttcatgtcgtggatgcctgggtttcaatcgatgcaaacgaggatcttattcaatgaagcttttagcagagggcttcgtatcatgcagattgtcactgggaagaaatcaaaaggcgatgtcgaagttgaaaaaagaaggtaaagcttcttatttacccaaacatcttttatgttctgtttgtttggaatcttaaattacaacaacactaatgcaaagcttttataacttgtgtaggtcttgaggtatatggtaatttaaaagttgctggtttgcggcgatgaggttagttttgtattcttataagttatgcttcttgtctgaataagaactcagacacccgtgttttgtcttcttcttattttaaaccaggtttttggagagctttggttgaggaagctatttgattagttcatcggttagtgggagaaacatatatatacatttgtcagtactttgttagagtgtgtggaaatggggacgactctgattctgattccttatgtggttattgtctgaaacgttacagcattttgtgaagtaggcttttgtgcaagatttgatatctttctctcattgtagagctttagagcattttttagtatatgtttaatctttgatttttctaatgtcatttgcattcatatttcac

SEQ ID NO: 5 - DNA, 8624 bp, Brassica oleracea
  source 1..8624: mol_type = genomic DNA
gtttctttttttttttggtcgaaattatattattgtttctctgagctgttaccattacattaacaatttacattctatccttttgatgaaaaatattataaaatgttaaaagaagttattagaaaaggagaggaaaacagggggagagcatggaggggtcccatgtgtgtttcggaaagcagcaaacatgactttgtaaagtcttgttttagcgtccaaagcggtctcactcgccgttcagcgagctttagctgttaaattttcttgaaataaatcgctccacttgttaaaaaaaaaaatgataactgtgtccatttcgactaatatctattttgtgtcatttttgcatataatattttttaatatttttgaaaataaatttaataaatagttttataaacaaaaaaaattgaaaaatagtaactattgataaaatacctatatgaacttagtagtattttttttcagttctaaaaatgtttaaatcataattttcagattatgttataaataaagcagaaatgacattctacgaagtagaaaacgaaatccattttttttcattgaatctacaatgtttagaatacgaaatcttcgtaaataagagtattctaaaaatatttagaatacacattccgcgcttaacctaccgatctaaaatctttagaaatcaaaatctacagattaatataaatctaaaacacgttgaaaccgacttctacagatttactgtaaatctaaaacatgtagaaatcaaaattctacacattactataattctaaaaacctatagaaaccgatttctacatattatctgtattctacggataagaaatcagttcttaaaaatatggaaacaaaatatttgagaatattcactttcatattttgaaaaaaatcgatttaaaaaaaacaaaaaaaacaaaaaaccttcttttcacgccgtcttctatattccattgattgttcacaaaattttcacattatttccaccatatcagtgtgaaattgagtgagttagggtttatgaacttgagactttgattttctccctttttgttcgtgaaggagatgagaaattatgagtttcatctcaaagaaatcgagtttaaagagttgaaatcgtgtttggtcggttcaaatcaagtgggaattaaaccggatataaccgaagaaaaccaggaaatcgatttggaatacttacctaggcacaagatcgatcggtctataattagagatcggttgatctgtatgaaatcgacttttgccgatcgagtgaaatggaccaggtcgatcagccgcgtttttttgttctgcataatgatcagaatcggtcaatccgtccgaccttgtaatttcggatcgatcgatcccgcttgatcgaacctattatttattatatttaagaattacaattttaaggattttattgccattttgaaaataattagtctaattgaacataaaatatataagattagtctaaaatgacatagttatcattttttgttctaaaaaaacaatttcccttttttatttttgtttctttcaacacacttgtattaataacaataatgatattgctaatcttgaacaaatcgtggattgtcttttcttccggtgatatcatccttagtcaaaacatctcaaattaaataagtatagagttgtgaatgtttttaaaagtttggcgtttgtatagatcactgtcagtgtcatgaatcattaggtgactgcaaatttttatatgacaaaaaagagagttgatacttgccattctcgagattttgaagtttttttcgtcgtcaacatacaaactcaacattttcgaaatcttggattaaaaataaaaatatggacaaaacgatacttattaattaattatgtactagcgtcttaacattattaatatagatataattataagaacaagaaacataaacatatatgcacaaagcctcaaagcaaatttaaataatgttacaaaacaagggatgtacttgttatgaaaaattaatatataaccattcttaacatatttttacgtaaaccttaaactttataaagaaaaatatgtaacattccggtgcgtggtatatagaaatatttttaaaaattgatttgactatttccattagcaaaatgcatttattttttcgatcatacatttatttaaaatttcagggttaaacgtgattaaaatggagtaataagaatatggatgatctaccagaaaatcatttacgttttaagtgagaccaaaatacggataaaaatcatgtgatgattgtatggttattaaacaattattttgaatttgaaaataattaactcatcaaattaaacctaaggaccgagtaagcggacgcagatagccgtaagcggttgggccgtcacaaaatttatgaccaacaagaaaatgaaactgattttagtggatgatatattttagaaagtaataaaatggttccagatttcaatacttcaatggtttttttatgctgactttcttttcctcttttacttacatgataaggaaacgagagaggttgaagaaacaaagaaaattcctaaggatttagaaatgtatcttcaaaaaatctaagtatttaccaagtaaaatcatacaaaataaggaaaaaaaaagaatttatttcccaatttggtttttaccggaaaaaaaattgttttaataaaatcttatgcaccaaatcatataagaacgaaccataacaaactttatttgaccattgtcattagtttattttatttatggtaatggatcttcaaataatttgaattaaattaaaaaaaagaataaaaaaagagaaacaaaaacgcggaaaggagagcccaaatcgtctccgtctgtcattgtcgcagtctctcacagctaaataaaagagaaaaacaaatcgcaacgcttcaatatctctctcccaatcgtttgaattagtcttcctcatcacaatacccctaagatccacctcacatgctactatgagcctccgccaccgcaccaccgtcccctctcaacccggacggcccccggcggcgggcgcaatcgacgaggagccctacaacatcatccccgtcaacaacctcctcgccgaccacccctccctccgctaccccgaggtccgcgccgccgccgccgccctcaaaaccgtcggagacctccgccgccccacctacgtccaatggcgcccccactacgacctcctcgactggctcgccctcttcttcggcttccagaaggacaacgtccgcaaccagcgcgagcacctcgtcctacacctcgccaacgcccagatgcgcctcacgccgccgccggataacatcgattccctcgatcccgccgtcgtccgccgtttccgccgcaagctcctcggtaactactcgagctggtgctcgtacctcgggaggaagtcgaacatctggatctcggatcggaaccccgattcgaggcgggagcttctctacgtcggcctctacctcctcgtgtggggggaggcggcgaatcttaggtttatgccggagtgtatctgttacatcttccacaatatggcctcggagcttaacaagatcctcgaggattgcctcgacgagagcacggggcagccgtattctcctagaatcacgggggagaatagtttcctaaacggcgtcgttaaacctatttacgagacgatcaaagctgagattaacgagagcaagaacgggacggagccgcattgtaagtggaggaactatgatgatattaacgagtacttttggacggataggtgtttcagtaaattgaaatggccgattgatttggggagcagtttcttcaagagtagtagagggagcggcgttgggaagacaggttttgtggagcggaggacgtttttttacctctacaggagctttgataggctttgggtgatgcttgctttgtttcttcaagctgctattatagttgcttgggaggagaagccgggtggagggtcggtgaggagtcagctctggaatgcgttgaagtcgacggatgttcaggtgaggcttttgactgtgtttttgacgtggagtgggatgagattactgcaggctgtgctggacgctggctcgcaacggccgcttatttctagagagaccaaacggctgtttttcagaatgctgatgaaggttgtagctgctacggtttggatcattgcttttattgttctctacacgaacatctggaagcagaggaagcaagacaggcagtggtccagagccgcgaatgacaagatctaccagttcctttacgctgtggtggctttcttggtccctgagatcctggctttggctctgtttatagtcccgtggataaggaactttctggaagagaccaattggaagatattctttgctttgacttggtggttccagggtaaaagctttgtgggtcgaggtttgagagaggggttggtggacaacatcaagtactcgactttctggatctttgtcctagcaacgaagttcacgttcagctacttcctgcaggttaagccaatgattaaaccctcgaagctgctatggaatttgaaggaggtggattatgagtggcatcagttctttggcaagagcaataggttttctgtcttgttattgtggctgccagtggtgttgatatacctgatggatatccaaatttggtacgcgatctattcttcgattgttggtgctgttgttgggctgtttgatcatctgggggagatcagggacatgggacagcttaggctgaggtttcagttctttgctagcgctattcagttcaacctaatgcctgaggaacaactcctgaatgctagaggatttggtaacaagcttaaggacgccattcataggtaagtctattgaagcatgttactgatatttctatataatttattatacagagtttgtctttacagtacaagctataggattttagttttgttaaagaagatttctccgcaatgaactcgacttttcacattgtaataacattgagtttgtgtactttatgcagattgaagctgaggtatggattggggcggccgtttaagaaactcgagtccaatcaggttgaggctaacaagtttgcgctgatctggaatgagataatcttagctttcagagaggaggatatagtctctgatcgagaagtagagctgctggagctgccaaagaattcctggaatgtgacagttatccgctggccgtgtttcctgttgtgcaacgagcttttgcttgcactgagccaggcgaaagagctggttgacgcacctgataaatggctgtggcacaagatatgcaagaatgagtacaggcggtgtgctgtggttgaggcatatgaaagcatcaaacatctgttgctctcaatcatcaaaattgacaccgaagaacataaaattgttacaattttctttcagatgattgaggtgtctattcagggtgagcagttcaccaagaccttcaaagtggacctattgccaaagatttatgagacgctacagaagttggttgggctgttgaatgatgagaaagtggatgttgggcgagtggtgaatggtctgcagtctatttatgagattgcaacacgacagttcttcatagaaaagaagacgactgaacagctatctaccgaggggttaactcctcatgatccagcctcaaagttactgtttcagaatgctgttaggcttcccgatgcaagcaatgaagacttcttccggcaggttaggcggttacacacaattctcacttctagggactctatgcacagcgtccctgtgaatctagaggcgagacggcggattgccttcttcagcaattcgctcttcatgaacttgcctcatgcacctcaggtggagaaaatgttggcgttcagtgttatgactccatactacagcgaggaagttgtatacagtaaagaacagctccgaaatgagactgaggatgggatttcaaccttgtattacctgcagacgatttatgccgacgaatggaaaaattttaaggaacggatgcgtagggaaggtataaagacagatgttgagttgtggacaaccaagctgagagagctcaggctttgggcttcctacagaggtcagactttggcacgtacagttcgaggaatgatgtactattacagggctcttaagatgcttgcttttctcgactctgcgtctgaaatggacattcgggaggatgctcaggagcttggttcaatgaggagttcgcagggaaatcgattggatggtgttgacgatgtaaatgaccgatcttctctaagcagagcaactagctctgtgagcatgctgtataaaggccatgagtatgggactgcattgatgaaattcacatatgtcgtggcgtgccaaatctatgggtctcaaaaagcgaagaaagagcctcaggcagaggaaattctgtatcttatgaagcaaaacgaagcccttcgtattgcatatgtggatgaggtacatgcgggcaggggagagactgagtattactccgttctggtgaaatacgatcacacgttggagagggaagtggagatattccgtgtgaagctacctggtccggtgaagctgggtgagggaaagccagagaaccagaatcatgcaatgatctttacccgtggtgatgctgttcagaccatagatatgaaccaggataattattttgaggaggctctcaagatgagaaatttgctccaggagtttaggcattatcatgggatcagaaaaccaactattcttggtgtcagagagcacatcttcacgggttctgtctcgtctctggcttggttcatgtctgctcaggagacaagtttcgtcactcttggtcagcgtgttctagccaacccgctgaaggtcagaatgcattatggtcaccctgatgtatttgacagattctggttcttgagtcgaggtggcatcagcaaagcttctagagttataaatatcagtgaggacatcttcgccgggtttaattgcacattgcggggcggtaacgtcacccaccacgagtatattcaggtagggaaatgttcatcatttggatattctaactaatttatacatcgacaacaatactataattccacttttttgttataacctttttgtgtgtgcatatgtattcaggttgggaagggtcgagatgttggattgaatcaaatatcaatgtttgaggctaaggtagccagtgggaatggagagcaggttcttagccgagatgtgtacaggttgggtcataggctcgatttcttcagaatgttatcatttttctacacaacggtggggtttttcttcaacacgatgatggtcattctcactgtctacgctttcctctggggccgggtttatcttgctctgagcggtgttgagaagtccgctctagcagacagcacagacaccaacgcagcgcttgctgtgatattgaaccagcagttcatcattcagcttggtctcttcacagctctgccaatgattgtggaatggtctctcgaggagggtttccttctcgcgatatggaacttcattcggatgcagattcagctttcttctgtcttctacacattctcaatggggaccagagctcactattttggccgaaccattctccacggtggagcaaagtacagagccactggacgtggatttgttgtcgagcacaagagtttcactgaaaactaccgtctatacgcgcgcagtcactttgtgaaggccatcgagcttgggctgatcctcatagtctacgctacgcacagtcccatcgccaaagactcattgatctatatagccatgactctcaccagctggttcctcgtgatttcatggatactagccccttttgtgttcaacccgtcaggtttcgactggcttaagacggtctacgacttcgaaggcttcatgaactggatctggtatcaaggcagaatctcaacgaagtccgaacagagctgggagatatggtggtatgaggaacaggaccacctgagaaccaccggtctaccaggaagaatcatggagataatcttggaccttcggtttttcttcttccagtacgggattgtataccagctcaaaatcgcaaacggatcaaccagcgttctcgtctacttactctcatggatatacatcttcgcagtgtttgtgttcttcctggtaatccaatacgcccgtgacaagtactcagcgagaaaccacatacggtacaggctcgttcagttcctcctgatcgtgtttggtacactggtgattgttgctctcctggagttcacgcatttcagcttcgtggatatcttcacgagtcttcttgcgttcgtcccaaccggctggggaatcttgctgatcgcacaggctttgaggcctgcgctgcagaagatcgggcttatctggaacgcggttatctcccttgctcggttatatgacatactgttcgggatagtcatcatggtccccgtagcgttcatgtcgtggatgcctgggtttcagtcgatgcaaacgaggatcttattcaatgaagcttttagcagagggcttcgtatcatgcagattgtcactgggaagaaatcaaaaggcgatgtcgaagttgaaaaaagaaggtaa

SEQ ID NO: 6 - DNA, 9270 bp, Brassica juncea
  source 1..9270: mol_type = genomic DNA
ctgtcagatttagtttcacaaaatctttgtaacttcgcggtttttgatatggaagttgctacaaaaactgacttgtgatattataatctttcggcaagaaaaatatataatactaatttcagaaagtattctgttgaattgttgatcaccaaatacacataaaccggcagatgttgacatgtttacgtgggatcactgggatagaagttttgcttctgtattagtatcgcgaaccggtttgtagtagcgaaaataacattattattttcagatttcatcatcgtcaaattcaacgttacatttgaacaggcttgtaaaaagtggacatgtggcatgagtaaaagataaagaaaattgtgagcctttttgttaatacgaaaaagccgaaaacgttattatttctatcatcggcaaatttaatgttaaatttgctccacatcattcagagggtatatgtatatttttctaatgcttcggtgaagcacatgcgaccatttgttgcgtcagaagtcagaacaaaaggaagattccatctaatggattataatcccacatgcccatttttaaaactagacaaaataacttataatagtcccataagagcattaagacaaactgaaccaaaaagaatcttaaatgctggtgaatctagtctcgaatgctgctgaacactcctgatattagaatttggcagaaaatattcatactaataacagtaaatacatttcaaaacaagaaaatagtagtagtaaataaaaacaattaatatgttattattgtttctcttagctgttaccattacattaacaatttacattcaatccttttaatgaaaaatattataaaatattaaaagaagttattagaaaaggagagggatatgggggggggagagcatggaggggtcccatgtgtgtttcgaaaagcagcaaacatgactttgtaaagtcttgttttagctagagttccaaaaaaaaaagagttcaaaaaaaaagaaaaaaaaaagtcttgttttagcgtccaaagcggtctcactcgccgttcagctgttaaattttcttgaaataaatcgctccacttgttttttatttttgtttctttcaacccacttgtattaataacaataatgatattgctaatcttgaacaaatcgtggattgtcttttcttccagtgatatcatccttagtcaaaacatctcaaattaaataaatatatagttgtgaattaaaaaaaaggtatagagtttataaaattagcatttgcgaatgtttttaaaagtttggcgtttgtatagatcactgtcagtgtcatgaatcattcggtgacagcaaatttgtatatgccaaaaaagagagttgatacttgccattctcgatattttgaattttttttcgtcgacatacaaactcaacattttcgaaatcttagattaaaaacaaaatggacaaaacgatacttattaatgaattatgtactagcgtctgaacattagtaacatagatataattataagaacaagaaacatatatgcacaaagcctcaaaccaaatttaaatagtgttacgaaacaagggatgtacttgttatgaaaaattaatgtataaccattcttagcattttttacctaacccttaaactttataaagaaaaatatgtaacatttcggtgtgtggtatataaaagtattttgaaaatcgatttgattatttctattattaaaatgtacttactttttttatcacacatttatttacaatttcagagttaaacatgattaagacaaagtagtgaaaatatagatgatctaccagaaaatcatttgctttctgagtgagatcaaaataaaggcaaaaataatgtgatgattgtatattaaacaattattttgaatttgaaaagaataactcatcgaatgaagcctatgaaccgagtaagcggtgaagcggttggaccgtcacaaaaattatgaccaacaagaaaataaaattgatattagtgaagggcaattgtcaataatagcaccttttgaagtttatgtctcaaaaatagcactagaaggagaaagtcacaaaaatgacattcattaaagggtaaaatatctataatacccttggtttaaaattaaataaacaaactaaaataaataaaaataaaaaaataaaaaaaataaaaataaaaaaaataaatttttttttatagtttcagattatatgttttcagattcgaaatttttataatttttttttaaaaaaaaattttaaatcttttttttatttttttttcagattttatttttataatttaaaaatactttttgaaactgtttttaaaatttttattttttattttattatttattatttataaaattttaaatcctaattccaaaaccccaccccttaactctaaaccctaatgtttggattaattaaccctaggggtataagtgtacattacctctttaatgaaacctatttttgtgactttgaaccttgagtgctactttgggaacaaaaacttggtttggtgctattctagtatttttctcattagtgaatgatatattttagaaagtaataaattggttccagatttcaatacatcaatgtttttctaatgctgacttgcttttcctctttttcttacatgataaggaaacgagagaggtcgaagaaacaaagaaacttcctaagcatttagcaacgcatcttcaaaaaatctagtatttaccaagtaaaatcatacaaaataaggaaaaaaagaagaatatatttcccaatttggttttcaccggaaaaaaaaaactgtcttaacaaaatcttaatgcaccaaatcatataagaactttatttgaccattgtcattagttttttccttatggtaatggatcttcaaataatttaaattaaattaaaaaaaaaaagaaaagagaaacaaaaacgcggaaaggagagcccaaatcgtctccgtctgtcattgtcgcagtctctaaaagagaaaaacaaatcgcaacgcttctctctctctccctatcgtttgaatcagtctctcaagatccaccaccaccacacatgctactatgagcctccgccaccgcaccgtcccctctcaacccggacggcccccggcggcgggcgcaatcgaggacgagccctacaacatcatccccgtcaacaacctcctcgccgaccacccctccctccgctaccccgaggtccgcgccgccgccgccgccctcaaaaccgtcggcgacctccgccgccccacctacgtccaatggcgcccccactacgacctcctcgactggctcgccctcttcttcggcttccagaaggacaacgtccgcaaccagcgcgagcacctcgtcctccacctcgccaacgcccagatgcgcctcaccccgccgccggacaacatcgattccctcgatcccgccgtcgtccgccgcttccgccgcaagctcctcggtaactactccagctggtgctcctacctcgggaggaagtccaacatctggatctcggatcggacccccgattcgcggcgggagcttctctacgtcggcctctacctcctcgtgtggggcgaggcggcgaatcttaggtttatgcctgagtgtatctgttacatcttccacaatatggcctcggagcttaacaagatcctcgaggattgcctcgacgagagcacggggcagccgtattctcctaagatcacgggggagaatagtttcctaaacggcgtcgttaagcctatctacgagactattaaagctgagattaacgagagcaagaacgggacggagccgcattgtaagtggaggaactatgatgatattaatgagtacttttggacggataggtgttttagtaaattgaaatggccgattgatttggggagcagtttcttcaagaacagcagaggtagcggcgttgggaagactggttttgtggagaggaggacgtttttttacctctacaggagctttgataggctttgggtgatgcttgctttgtttcttcaagctgctattatagttgcttgggaggagaagccgggtggagggtcggtgacgagtcagctctggaatgcgttgaagtcgacggatgttcaggtgaggcttttgactgtgttcttgacgtggagtgggatgaggttgttgcaggctgtgttggacgctggctcgcaacggtcgcttatttctagagagaccaaacggctgtttttcagaatgttgatgaaggttgtggctgctacggtttggatagtagcgtttattgttctctacacgaacatctggaagcagaggaagcaagataggcagtggtccagagccgcgaatgataagatttatcagttcctttacgctgtggtggctttcttggtccctgagatcctggctttggctctgtttatagtcccgtggataaggaactttctggaagagacgaattggaagatattctttgctttgacttggtggttccaggggaaaagctttgtgggtcgaggtttgagagaggggttggtggacaacatcaagtactcgactttctggatctttgtccttgcaacgaagtttacgttcagctacttcctgcaggttaagccaatgattaaaccctcgaagctgctatggaatttgaaggaggtggattatgagtggcatcagttctttggcgagagcaataggttttctgtcttgttattgtggctgccaatggtgttgatatacctgatggatatccaaatttggtacgcgatctattcttcgattgttggtgctgttgttgggctgtttgatcatctgggggagatcagggacatgggacagcttaggctgaggtttcagttctttgctagcgctattcagttcaacctaatgcctgaggaacaactcctgaatgctagaggatttggtaacaagcttaaggacgccattcataggtaagtctattgaagcatgttactgatatttctatataatttactatatagtttgtctttacagtacaagctatgggattttagttttgttaaagcagatttctccgcaatgaactcgacttttcacattgtaataacattgagtttgtgtactttatgcagattgaagctgaggtatggattggggcggccgtttaagaaactcgagtccaatcaggttgaggctaacaagtttgcgctgatctggaatgagataatcctagctttcagagaggaggatatagtctctgatcgagaagtagagctgctggagctgccaaaaaattcctggaatgtgacagttatccgctggccgtgttttctgttgtgcaacgagcttttgcttgcactgagccaggcgaaagagctggttgacgcacctgataaatggctgtggcacaagatatgcaagaatgagtacaggcggtgtgctgtggttgaggcatatgaaagcatcaaacatctgttgctctcaatcatcaaaattgacaccgaagaacataaaattgttacaattttctttcagatgattgaggtgtctattcagggtgagcagttcaccaagaccttcaaagtggaccttttgccaaagatttatgagacactacagaagttggttgggctgttgaatgatgagaaagtggatgttgggcgagtggtgaatggtctgcagtctatttatgagattgcaacacgacagttcttcctagaaaagaagacgactgaacagctatctactgaggggttaactcctcatgatccagcctcaaagttactgtttcagaatgctgttaggcttcccgatgcaagcaatgaagacttcttccggcaggttaggcggttacacacaattctcacttctagggactctatgcacagcgtccctgtgaatctagaggcgagacggcggattgccttcttcagcaattcgctcttcatgaacttgcctcatgcacctcaggtggagaaaatgttggcgttcagtgttatgactccatactacagcgaggaagttgtatacagcaaagaacagctccgaaatgagactgaggatgggatttcaaccttgtattacctgcagacgatttatgccgacgaatggaaaaattttaaggaacggatgcggagggaaggtataaagacagatgttgagttgtggacaaccaagctgagagagctcaggctttgggcttcctacagaggtcagactttggcacgtacagttcgaggaatgatgtactattacagggctcttaagatgcttgcttttcttgactctgcgtctgaaatggacattcgggaggatgctcaggagcttggttcaatgaggagttcgcagggaaatcgattggatggggtggacgatgtaaatgacggatcttctctaagcagagcaactagctctgtgagcatgctgtataaaggccatgagcatgggactgcattgatgaaattcacatatgtcgtggcgtgccagatctatgggtctcaaaaagcgaagaaggagcctcaggccgaggaaattctgtatcttatgaagcaaaacgaagccctccgtattgcatatgtggatgaggtgcatgcgggcagggaagagactgagtattactccgttctggtgaaatacgatcacacgttggagaaggaagtggagatattccgtgtgaagctacctggtccggtgaagctgggtgagggaaagccagagaaccagaatcatgcaatgatctttacccgcggtgatgctgttcagaccatagatatgaaccaggataattattttgaggaggctctcaagatgagaaatttgctccaggagtttaggcattaccatgggatcagaaagccaactattcttggtgtccgggagcacatcttcacgggatctgtctcgtctctggcttggttcatgtctgctcaggagacaagtttcgtcactcttggtcagcgtgttctagccaacccgctgaaggtcagaatgcattatggtcaccctgatgtatttgacagattctggttcttgagtcgaggtggcatcagcaaagcttctagagttataaatatcagtgaggacatcttcgccgggtttaattgcacattgcggggcggtaacgtcacccaccacgagtatattcaggtagggaaatgttcatcatttggatattctaactaatttatacatcgacaacaatactataattccactttttttttgttataacctttttgtgtgtgcatatatgtattcaggttgggaagggtcgagatgttggattgaatcaaatatcaatgtttgaggctaaggtagccagtgggaatggagagcaggttcttagccgagatgtgtacaggctgggtcataggctcgatttcttcagaatgttatcatttttctacacaacggtggggtttttcttcaacacgatgatggtcattctcactgtctacgctttcctctggggccgggtttatcttgctctgagcggtgttgagaagtccgctctagcagacagcacagacaccaacgcagcgcttgctgtgatattgaaccagcagttcatcattcagcttggtctcttcacagctctgccaatgattgtggaatggtctctcgaggaaggtttccttctcgcgatatggaacttcattcggatgcagattcagctttcctctgtcttctacacattctcaatggggaccagagctcactattttggccgaaccattctccacggtggagcaaagtacagagccactggacgtggatttgttgtcgagcacaagagtttcactgaaaactaccgtctatacgcacgcagtcactttgtgaaggccatcgagcttgggctgatcctcatagtctacgctacgcacagtcccatcgccaaagactcattgatctacatagccatgactctcaccagctggttcctcgtgatttcatggatactggccccttttgtgttcaacccgtcaggattcgactggcttaagacggtctatgacttcgaaggcttcatgaactggatctggtatcaaggcagaatctcaacgaagtccgaacagagctgggagatatggtggtatgaggaacaggaccacctgagaaccaccggtataccaggaagaatcatggagataatcttggaccttcggtttttcttcttccagtacgggattgtataccagctcaaaatcgcaaacggatcaaccagcattctcgtctacttactctcatggatatacatctttgcagtgtttgtgttcttcctagtgatccaatacgcccgtgacaagtactctgcgagaaaccacatacggtacaggctcgtccagttcctcctgatcgtgtttggtacactggtgattgttgctctcctcgagttcacgcatttcagcttcgtggatatcttcacgagtcttcttgcgttcgtcccaaccggctgggggatcttgctgatcgcacaggctttgaggcccgcgctgcagaagatcgggcttatctggaacgcggttatctcccttgctcggttgtatgacatactgttcgggataatcatcatggttcccgtagcgttcatgtcgtggatgcctgggtttcaatcgatgcaaacgaggatcttattcaatgaagcttttagcagagggcttcgtatcatgcagattgtcactgggaagaaatcaaaaggcgatgtcgaagttgaaaaaagaaggtaaagcttcttatttacccaaacatattttatgttctgtttgtttggaatcttaaattacaacaacactaatgcaaagcttttataacttgtgtaggtcttgaggtatatggtaatttaaaagttgctggtttgcggcgatgaggttagttttgtattcttataagttatgcttcttgtctgaataagaactcagacacccgtgttttgtcttcttcttattttaaaccaggtttttggagagctttggttgaggaagctatttgattagttcatcggttagtgggagaaacatatatatatacatttgtcagtactttgttagagtgtgtggaggtggggacgactctgattctgattccttatgtggttattgtctgaaacgttacagcattttgtgaagtaggcttttgtgcaagatttgatatctttctctcattgtagagctttagagcattttttagtatatgtttaatctttgattttctaatgtcatttgcattcatattcacatcttctctgcttcttcgttgtctgaaaccagttttcagatgcttatccattgtcca

SEQ ID NO: 7 - DNA, 6389 bp, Brassica juncea
  source 1..6389: mol_type = genomic DNA
tatcattgtcgcagtctctctcacagctaaaaggaaaacagatcgcaacgcttcaatatctctctctctccattgttttgaattgaatcagtctcctcacccttctccaagatccaccacaccacatgccactatgagcctccgccaccgcaccgtcccatctcaaaccggacggccgtcggcggcgggaatcgaggaggagccctacaacatcatccccgtcaacaacctcctcgccgaccatccttctctccgttaccccgaggtccgcgccgccgccgccgctctcaaaaccgtcggcgacctccgccgtcctccctacgtccaatggcgtcctcactacgatctcctcgactggctcgccctcttcttcggcttccagaaggataacgtccgcaaccagcgcgagcacatggtgctccacctcgccaacgctcagatgcgtctcacgccgccgccggataacatcgattccctcgattcgacggttgtccgtcgctttcgccggaaactcctcggaaactactcgagctggtgctcttatttagggaagaaatcgaacatctggatctcggatcggaaccctgattcgaggcgggagcttctctacgttggcctctacctcctcgtgtggggcgaggcggcgaatcttaggtttatgcctgagtgcatctgttacatcttccataacatggcctcggagcttaataagattctggaagattgcctcgatgagaacacggggcaaccctatctgcctactctctcgggggaaaacgctttcctaaacggcgtcgttaaacctatttacgaaactatcaaagctgagattgatgagagcaagaacgggacggagccgcattgtaagtggaggaactatgatgatattaatgagtatttctggacggataggtgtttcagtaaattgaagtggccgcttgatctgggaagcagtttcttcaagagtagtagagggaaaagcgttgggaaaaccggttttgtggagcgcaggaccttcttttacctctacaggagctttgataggctttgggtgatgcttgcgttgttccttcaggccgccattataattgcttgggaggaaaagccggatagagggtcggtgacagggcagctgtggaatgccttgaagtccagagatgtccaggtgaggcttttgacagttttcttgacgtggagtgggatgagactactgcaggctgtgctggacgctggttcgcaacggtctcttatttctagagagaccaaacggctctttttcagaatgttgatgaaggttgtagctgccacagtttggataatagcttttattgtactctacacgaacatctggaagcagaggaagcaagacagacagtggtccagagccgcgaatgacaagatctaccagttcctttacgctgtggtggccttcttgatccctgagatcctggctctggccctgtttataatcccgtggattaggaactttctggaagagagcaattggaaaatattctttgctttaacttggtggttccagggtaaaagctttgtgggtcgaggtttgagagagggtttggtggacaacatcaagtactcgacgttctggatcttcgtcctagcaacaaagttcacattcagctacttcctacaggttaagccaatgattaaaccctcgaagctgctgtggaacttaaaggaggtagattatgagtggcatcagttctttggcgagagcaataggttttctgtcttattattgtggctgccagtggtgttgatatacctgatggatatccaaatttggtacgcaatctattcttcgattgttggtgctgttgttgggctgtttgatcatctgggggagatcagggacatgggacagcttaggctgaggtttcagttctttgctagcgctattcagttcaacctgatgcctgaggaacaactcctgaatgctagaggctttggtaacaagcttaaggacgccatccataggtaagtctgtggaagcatgttactgatttcctttagagtttaatgtacagagtttgtctttacggtacaagctatataattttagttttgttatagcagattctcgtaacttgactttttaacattgttataaccttgagtttgtgtactttatgcagattgaagctgaggtatggatttgggcggccgtttaagaaactcgagtctaatcaggttgaggccaacaagtttgctttgatctggaatgagataatcttagcttttagagaagaggatattgtctctgatcgagaagtagagctactggagctgccaaagaattcctggaatgtgacagttatccgctggccgtgtttcctgctgtgtaacgagcttttgcttgcactgagccaggcgaaagagctggttgatgctcctgataaatggctgtggcacaagatatgcaagaatgagtacaggcgttgtgctgtggttgaggcatacgacagcatcaaacatctgttgctctcgatcatcaaaatcgacactgaagaacataaaatcatcacggttttctttcagatgattaaggtttctattcagggagagcagttcaccaagaccttcaaagtggatcttctgccaaagatttacgagacactacagaagttggttgggctgttgaatggtgaggaaccggatatcgggagagtggtgaatgttctgcagtctatatatgagattgcaacacgacagttctttatagaaaagaagacaactgaacagctatctactgaaggattaactcctcatgatccagcctcaaagttactgtttcagaacgctgttaggcttcccgatgcaagcaatgaagacttcttccggcaggtgaggcggttacacacaattctcacttctagggactctatgcacagcgtccctgtgaatctagaggcgagacgtcggattgccttcttcagcaattcgctcttcatgaacttgcctcatgcacctcaggtggaaaaaatgttggcgttcagtgttatgactccatactacagcgaggaagttgtatacagcaaagaacagctcaaaaatgagactgaggacgggatttcaaccttgtattacctgcagacgatttatgctgacgaatggaaaaattttaaggaacggatgcgtagggaaggtataaagacagatgatgagctgtatacaaccaagctgagagagctcaggctttgggcttcctacagaggtcagactttggcacgtacagttcgagggatgatgtactattacagggctcttaagatgcttgcttttcttgactctgcgtctgaaatggacattcgggaggatgctcaggagcttggttcaatgaggagttcgcagggaaatctgggcggtcgatcgaatggggttgacgatgtaaatgaccgatcttctctaagcagagctactagctccgtgagcatgctgtataaaggccatgagcatgggactgcattgatgaaattcacatatgtcgtggcgtgccagatctatgggtctcaaaaagcgaagaaggagcctcaggcagaggaaattctctatcttatgaagcaaaatgaagccctccgtattgcgtatgttgatgaggtgcatgcaggcaggggagagaccgaatattactcagttctggtgaaatacgatcacactttggagaaggaagtggagatattccgtgtgaagctacctggtcccgtgaagctgggtgagggaaagccagagaaccagaatcatgcaatgatctttacccgtggtgatgctgttcagaccatagatatgaaccaggataattattttgaggaggctctcaagatgagaaatttgctccaggagtttagacattatcatgggatcagaaaaccaactattcttggtgtccgagagcacatcttcactggctctgtctcgtctctggcttggttcatgtccgctcaggagactagtttcgtcactcttggtcagcgtgttcttgctaacccgctgaaggtcagaatgcattatggccaccccgatgtatttgacagattctggttcttgagtcgaggtggcatcagcaaagcgtccagagtcataaatatcagtgaggacatcttcgctgggtttaactgcacattgcggggcggtaacgtcacacaccacgagtatattcaggttggtaactattcattatttggttatttctaactaatttatactgcgacagcaatcctatatttccatatttcttttgttataaccatgcaacttaacgttcattgtatctgagtgtcaatgtaaatttcataacccctgtttttgtgcatatattcaggttgggaagggtcgagatgttggattgaatcaaatatcaatgtttgaggcgaaggtagccagtgggaacggagagcaggttcttagccgagatgtgtacaggctgggtcatagactcgatttcttcagaatgttatcatttttctacacaacggtcgggtttttcttcaacacgatgatggtcattcttaccgtttacgctttcctatggggccggatttatcttgctctgagcggtgttgagaagtccgctctagcagacagtacagacaccaacgcagcgcttgcggttatattgaaccagcagttcatcattcagctcggtctcttcacagcactgccaatgattgtggaatggtctctcgaggaaggtttccttcttgcgatatggaatttcatccggatgcagattcagctttcttctgtcttctacacattctcaatggggaccagagctcactattttggccgaaccatcctccacggtggagcaaagtacagagccactggacgtggatttgttgtcgagcacaagagtttcactgagaactacagactgtatgcacgcagtcactttgtgaaggccatcgagcttgggctgatcctcatagtctacgctacgcacagtcccatcgccaaagactcattgatctatatagccatgactctcaccagctggttcctcgtgatatcatggatactggctccatttgtgttcaacccgtcaggtttcgactggcttaagacggtctatgacttcgaaggtttcatgaactggatctggtatcaaggcagaatctcaacgaaatccgaacagagctgggagatatggtggtacgaggaacaggaccacctgagaaccaccggtataccaggaagaataatggagataatcttggaccttcggtttttcttcttccagtacgggattgtataccagctcaaaatcgcaaacggatcaaccagcattctcgtctacttgttgtcgtggatatacatctttgctgtgtttgtgttcttcctggtaatccaatacgcccgtgacaagtactctgcgaaaaaccacatacggtacaggcttgtccagttcctcctgatcgtgtttggtattctggtgatcgttgctctgctggagttcacgcatttcagcttcgtggatatcttcacgagtcttcttgcgttcgtcccaaccggctggggaatcttgctgatcgcacaggctttaaggcctatgctgcagaagttcaggcttatctggaacgctgttgtctcccttgctcggttatatgacatactgttggggatactcatcatggttcccgtagcattcatgtcatggatgcctgggtttcagtcaatgcaaacgaggatcttattcaatgaagcttttagcagagggcttcgtatcatgcagattgtcactgggaagaaatcaaaaggcgatgtctaagttgaaaatgaaagaaggtaaagctctttatttactcaaacatcttttatgttctgtttgtttggaatcctaagattacaacaaaaccaatgcaaagctttataacttgcgtaggtcataataaggtacatggtaatttaaagttgttggtttgcggcgttgagatcagttggaggttagttttctcgagacatggtattctataagttattgcttcttgtctgaataagaactcaaaagaaaaaccatgtgttgttgttgttgtcttcttcttaaagcaggtgtttggagagcttttgttgaggaatctggaagttgggttagatcatgggttagcgggtgaaatatatattgtcagtactttgttagtgtgtggaaatgggactctgattcttgttgtctgaaacgatacagcattttgtgaagtagggcttttgtgaaagatttgtttctctttctctctcagtgtagagctttagagcattttttagtatatgtttaatctttttattttctaatgtcatttgcattcatatctcacgtcttcctcgttggtctgaaaccggttttgagatgcttatccattgtccacttctctatg

SEQ ID NO: 8 - DNA, 9343 bp, Raphanus sativus
  source 1..9343: mol_type = genomic DNA
caaacgatcatagaaatgtacctgtaattagtcaactgttcaaagagcttaatgcattgctccttatcaatctgcccggttttctgtcataaacatgaaatagaatacaacgtaaacacatatgtttagctatgtggtaactaacagggagcttccctgtatatatctgtaggaggtaaaaatcattttgaatggagtaacttacgtctttgtctataagaccaaaggctttctccagcattcttctcttcatttgatccattccagatacttgctttgcgagctacaaaaataacaaatatgataccacgctagtgcggtcgtttttagttttaacatacaaaagatcaagttttgcaataaacctgttctttgaaactgtcataaacaacggcaagaatcaagttcgtgacaaagtagacgccaattagtacgtagagcacgaagaacaacgaagaccagcgtgaagacctatacaaaaaaaaaaaagaacaaatcagtcgcccaaaacactggatgtaactcatttcaccatataaacttacttgtaagcacgaatccagacatcaggattgttggatgttgtgaacaaaataaacatctggtaaagagttgcaccgtaagacgtgaagaccgtgagtccttgttgtgtatcctcaaacataacaaaagcaatccaactggcaaagagaaggaacagcatccatagagcctgtggagatattcaagaagtgaaagcatagaaggacaatcaatacgagttcatcactgttctgaaagtcaaactcgattgggaagaccactgaccaagatattcaagtatgtgccaagcattccagaaagaaggacgaggctgtctcgaagttccctgtacagaaattttaagaaacacagtttttagacaagaagataatataaaacaaaagtgcactttcatcgtaaatggcattttggattgagacaagttgatagaaaagaagcataaatatgtgttgataccttatgctgaggatgaatatgataactctgacatatggggcgattctaaaaggaagaaaatcgaaagccactggagacaagtatagaatgtcaacgagcacatcaacaatcaaaactaccacgcaagcaacctggaatcaggaagaagaagacatttattgtgttaaaagttatgaaatcaatatcttaagttctgtccaacattcaacaaatagaaaagaaaaaaaaaagaaacagtgaagaagacttatgtaggggagaataccttcactaggttaaggcggcttgtccaaaagatacgggacccttcataggagattgggaaaaaagtatgtacaagtagtataaccagggtaagtacctgtttggagaaagcaaaaatataagaatttcagtacaatgagaaaggatcctggctagtccgaacgataagataacgagtatataaatattagcatctacttaaacgagatcaactagttttcacaaaagtgtgtaatgaatctcaagccttgaactttcaagtggatgcatataagaatatgtcagtacagtgagaaaggatcctggctagtctagtcccaacaatatacaccatggaagataagacgagtatgttaataaaattaacaacttcttaaacgagatcaacgagtcttgaatctttcaaaagtgggttaatatgaatctggtgtgcctaattgcactaaaatctatttgcatctacagcgaaaatgaaaggccagctacttgcctcaaagataatggattctgcattggtcaagtagggtaactccccaaggtaatagtaatctctgtctttgcaagacggcgtaggcttattttcacaccacaatggttgctgcaaaaagacaggacaagaaagactgtcacacttttttctattttcttttaaaagtattttcttttgggggggttggggggggggcaaaaggttgctgacctcaaagaagttaatcaaaatgagagcgaaatagttgagagaccagatgagatctaatcgtgtgtagataaagtagtacttggcagactctccgaagctggactggtcaagtatttgctcaggtagacctataccatcttcagcctacatacatacagcaaaataaataaataaataaataaaaaggttctcaaaatcagcaaaaaagacaaagaaaccgaacattttctattgctatattcgtaacttattatcaggttaaagaaacaaatcattttgaacaaaaaaaaaaaaaaaagaaacaaatcatattctgagcaattattcagaataaacgatttggacttgtcagactgattctattcactgataaattgagaaatctccctcaagggagttatgccatcatgtcacagtcagtcggacaaagatccatgaattttatcagaacaagaagaagacaaatatagttagggagttgagagatagaaagagaaccagatcgacgagagcagcagctttctgaaaggtggtaccatgagcgatagcttctgatctacgaacaatccgatccgtaccaccaccacgactctctctacctatcaaaggatcttccattttttttttcttcaaaaggatcgaaatggaaagcagaagaccaaggaccttatgtagtacctttctttctttctttctgtcagtttattgttggctacgaattttaatataatgatacagatcacaagaagaagatagtgatgatggcccagaagtagttgaatttttaaaataaattaaattttccaagtgatattagatcttgccgacaaacacgttggggtccctttctcaatttgtaactttgtggatcaggatctaagtagattggtcaaaactgagagagtggtgttgtggtccgaataaaactgattaaagaataagactgcagagactaacaaacagaagaaacagatacatagagaagtggacaatggagaagcatctcaaaactggtttaacaagcagagaagaagatgtgaaatatgaatgcaaaatgacattagaaaatcaaagattaaacatatactaaaaagaaagtactctaaagctctacaatgagagagaaagagaagaaatctgaacacaaaagccctacttcacacaaaatgctgtaacgtttcagacaataacaccatacaagaatcagaatcagagtcttccccccttcccccacactctaacaaagtactgacaaatgtatatatatatgtttcccccactaaccgatgctctaaccagataaccaacttccaaattcgtccacaaaagctctccaaaaacctgtttcaagcacaagacagaacaaaagatgggtttatttgagttcttcttcgcacaccaaggataacttaaaaaaaattccatctctcgagaaaactaactaacctccaaatgatcaccatcgccgcaaaccaacagctttttcaagttaccatttaccatacgacctacacaagttataaagcttcgcattggtcttgttgtaaatcttaggattccaaaacaaacaggatattaaagatgtttcagtaaataaaagagctttaccttcttctttcttcaacttagacatcgccttttgatttcttcccagtgacaatctgcatgatacgaagccctctgctaaaggcttcattgaataagatccttgtttgcattgattgaaacccaggcatccacgacatgaacgctacgggaaccatgatgagtatcccgaacagtatgtcatataccctagcaagggagacaaccgcgttccagataagcctaaacttcgtcagcgctggccttaaagcctgtgcgatcagcaagattccccatccggttgggacgaacgcaagaagactcgtgaagatatccacgaagctgaaatgcgtgaactctagcagagcaacaatcaccagaataccaaacacgatcaggaggaactgaacgagcctgtaccgtatgtggtttctcgcagagtacttgtcacgggcgtactggattatcaggaagaacacaaacactgcaaagatgtatatccatgacaacaagtagacgagaatgctggttgatccgcttgcgattttgagctggtaaacaatcccgtactggaagaagaaaaaccgaaggtccaagattatctccacaactcttcctggtataccggtggttctcaggtggtcctgttcctcataccaccatatctcccagctctgttccgatttcgttgagattctgccttgataccagatccagttcatgaagccttcgaagtcatagaccgtcttaagccagtcgaatcctgacgggttgaacacaaatggggccagtatccatgatatcacgaggaaccaactggtgagagtcatggctatgtagatcaatgagtctttggcgatgggactgtgcgtagcatagactatgaggatcagcccgagctcgatggccttcacaaagtgactgcgtgcatagagtcggtagttctcggtgaaactcttgtgctcgacaacaaatccacgtccagtggctctgtactttgctccaccatggagaatggttcgaccaaaatagtgagctctggtccccattgagaatgtgtagaagacagaggaaagctgaatctgcatccgaatgaaattccatatagctagaaggaaaccctcctcgagagaccattccacaatcattggcagggcagtgaacagaccaagctgaacgatgaactgctggttcagtatcacagcaagcgctgcgttggtgtctgtactgtctgctagagcggacttctcaacaccgctcagcgcgagataaacccggccccagaggaaagcgtaaaccgtaagaatgaccatcatcgtgttgaagaaaaacccgaccgttgtgtagaaaaatgataacattctgaagaaatcgagcctatgacccagcctgtacacatctcggctaagaacctgctctccattcccactggctaccttagcctcaaacattgatatttgattcaatccaacatcccggcccttcccaacctgaatatatgtacaaaaaacaagggttatgcaatttacattgaagaaacaaggaacgttaagttgcatggttataacaaaaaaaaaaattgaactataggatttctgtcgcagtataaattagttagaaatatcaaaataatgaacattaccaacctgaatatactcgtggtgggtgacgttaccgcctcgcaatgtgcaattaaacccggcgaagatgtcttcactgatatttatgactctggaagctttgctgataccacctcgactcaagaaccagaatctgtcaaaaacatcggggtgaccataatgcattctgaccttaagcgggttggcaagaacacgctgaccaagagtgacaaaactagtctcctgagcagacatgaaccacgccagagacgagacagagcccgtgaagatgtgctcccggacaccgagaatagttggctttctgatcccatgagattttctaaactcctggagcaaatttctcatcttgagagcctcctcaaaataattatcctggttcatatctatggtctgaacagcatcaccacgggtaaagatcattgcatgattctggttctctggctttccctcacccagcttcaacggaccaggcagcttcacacggaatatctccacttccttctccaacgtgtgatcgtatttcaccagaactgagtaatactctgtctctcccctgcccgcatgcacctcatccacatacgcaatacggagggcttcattttgcttcataagatacagaatttcctctgcctgaggctccttctttgctttttgagacccatagatctggcacgccacgacatatgtgaatttcatcaatgcagtcccatgctcatggcctttatacagcatgctcacggagctagttgctctgcttagagaagatccaccatttacatcgtcaaccccatccagtcgaccatttccctgcgaactcctcattgaaccaagctcctgagcatcctcccgaatgtccatttcagacgcagagtcaagaaaagcaagcatcttaagagccctgtaatagtacatcattcctcgaactgtacgtgccaaagtctgacctctgtaggaagcccaaagcctgagctctctcagcttggttgtccacaactcaacatctgtctttataccttccctacgcatccgttccttaaaatttttccattcgtcagcataaatcgtctgcaggtaatacaaggttgaaatcccatcctcagtctcgtttttgagctgttctttgctgtatacaacttcctcgctgtagtatggagtcagaacactgaacgccaacattttctccacctgaggtgcatgaggcaagttcatgaagagcgaattgctgaagaaggcaatccgccgtctcgcctctagattcacagggacgctgtgcatagagtccctagaagtgagaattgtgtgtaaccgcctaacctgccgaaagaagtcttcattgcttgcatcgggaagcctaacagcgttctgaaacagtaacttggaggctggatcatgaggagtcaacccctcattagatagctgttcagttgtcttcttctctatgaagaactgtcgtgttgcaatctcataaatcgactgcaaaacattcaccactcgctcaatatctggcttctcagcattcagtagcccaaccaacttctgaagtgtctcgtacatctttggcagaaggtccactttaaaggtcttggtgaactgctcaccctgaatagagacctcaatcatctggaagaagatcgtaatgattttatgttcttcggtgtcaatcttgatgattgagagcagcagatgtttgatgctgtcatatgcctcaacaacagcacaacgcctgtactcattcttgcatatcttgtgccacagccatttatcaggagcatcaaccagctctttcgcctggctcagtgcaagtaaaagctcgttgcacagcaggaaacacggccagcggataactgacacattccacgaattctttggcagctccagtagctctacttctcgatcagagactatatcctcttctctgaaagctaagattatctcattccagatcaacgcaaacttgttggcttcaacctgattagactcgagtttcttaaacggccgcccaaatccatacctcagcttcaatctgcataaagtacacaaactcaaggttattattatgttgaaaactcgaattccaagcttgtaccgtaaagacaaactctgtatagtaaactataaatataggaatatgcttgcacagacttacctatgaatggcgtccttaagcttgttaccaaagcctctagcattcaggagttgttcctcaggcattaggttgaactgaatagcgctagcaaagaactgaaacctcagcctaagctgtcccatgtccctgatctcccccagatgatcaaacaacccaacaatagcaccaacaatcgacgaatagattgcgtaccaaatttggatatccatcaggtatatcaacaccactggcagccataataacaagacagaaaacctattgctctcgccaaagaactgatgccactcataatctacctcctttaagttccatagcagcttcgagggtttaatcattggtttaacctgcaggaagtagctgaaaatgaacttcgttgctaggacaaagatccagaacgccgagtacttgatgttgtccaccaaaccctctctcaaacctcgacccacaaagcttttaccctggaaccaccaagttaaagcaaagaatattttccaattgctctcttccagaaagttccttatccacgggattataaacagagccaaagccaggatctcagggaccaagaatgccaccacggcgtaaaggaattggtagatcttgtcattcgcggctctggaccactgtctatcttgcttcctctgcttccagatgttcgtgtagagaacaataaaggctataatccaaaccgtggcagctacaaccttcatcaacattctgaaaaacagccgtttggtctctctagaaatgaggggccgttgcgaaccagcgtccagcacagcctgcagtagtctcatcccactccacgtcaagaaaactgtcaaaagcctcacctgaacatctctcgacttcaaggcattccacatctgctttgccaccgaccctctatccggcttctcctcccaagcaactataatggcggcttgaaggaacaaagcaagcatcacccaaagcctatcaaagctcctgtagagataaaaaaacgtcctccgctccacaaaaccggtcttcccaacgctcttccctctactattcttgaagaaactgctccccaaatcaagcggccatttcaacttactgaaacacctatccgtccagaaatactcattaatatcatcatagttcctccacttacaatgcggctccgtcccgttcttgctctcattaatctcagctcggatcgtctcgtaaataggtttaacgacgccgtttaggaaagcgttctccccagagagagtaggcgtataaggctgccccgtgttctcgtcgaggcaatcctccaacaccttgttaagctccgaggccatattgtggaagatgtaacagacgcactcgggcatgaacctaagattcgcggcctcgccccacacgaggaggtagagaccgacgtagagaagctcccgcctcgaatcggggctccgatccgagatccagatgttcgatttcctcccgaggtaggagcaccagctggagtagttcccgaggagcttgcggcggaagcggcggacgacggcgggatcgagggagtcgatgttgtcggggggaggggagaggcgcatctgggcgttggcgaggtggaggacgacgtgctcgcgctggttgcggacgttgtccttctggaagccgaagaagagggcgagccagtcgaggaggtcgtagtgagggcgccattggacgaagggaggacggcggaggtctccgacggttttgagagcggcggcggcggcgcggacctcggggtagcggagggaagggtggtcggcgaggaggttgttgacggggatgatgttgtagggctcctcctcggttccccccgccgacggccgtccggtttgagatgggacggtgcggtggcggaggctcatagtagcatgtggtggatcttggagatggtgtgaaggaggaggagactgattcaaaggatgtggagagagagagagagagagagagagagagagagagagagagagattgaattgaagcgttgcgatatgtttttctcttttagct

SEQ ID NO: 9 - DNA, 23 bp, Brassica sp.
  source 1..23: mol_type = genomic DNA
acacgaacatctggaagcagagg

SEQ ID NO: 10 - DNA, 22 bp, Brassica sp.
  source 1..22: mol_type = genomic DNA
gaaagccaccacagcgtaaagg

SEQ ID NO: 11 - DNA, 23 bp, Arabidopsis thaliana
  source 1..23: mol_type = genomic DNA
acgaaaccgacgaacaaccgcgg

SEQ ID NO: 12 - DNA, 23 bp, Arabidopsis thaliana
  source 1..23: mol_type = genomic DNA
tattgattctctcgattccgcgg

SEQ ID NO: 13 - DNA, 23 bp, Arabidopsis thaliana
  source 1..23: mol_type = genomic DNA
gaacgccattgaacatacggcgg

SEQ ID NO: 14 - DNA, 23 bp, Arabidopsis thaliana
  source 1..23: mol_type = genomic DNA
gattgcctcgatgagaacaccgg

SEQ ID NO: 15 - DNA, 19 bp, Synthetic construct
  source 1..19: mol_type = other DNA
cgccgtctcagagctacaa

SEQ ID NO: 16 - DNA, 20 bp, Synthetic construct
  source 1..20: mol_type = other DNA
ggcggcttgaaggaacaaag

SEQ ID NO: 17 - DNA, 48 bp, Synthetic construct
  source 1..48: mol_type = other DNA
gtcgacctgcaggcatgcctgtcttaaatggacatttgtagtaacaaa

SEQ ID NO: 18 - DNA, 40 bp, Synthetic construct
  source 1..40: mol_type = other DNA
aagttctctcctttactgacatcgcctttttgatttcttc

SEQ ID NO: 19 - DNA, 20 bp, Synthetic construct
  source 1..20: mol_type = other DNA
cctgttccaaaggtcctgca

SEQ ID NO: 20 - DNA, 20 bp, Synthetic construct
  source 1..20: mol_type = other DNA
tgtcataccacttgtccgcc

SEQ ID NO: 21 - DNA, 38 bp, Synthetic construct
  source 1..38: mol_type = other DNA
tatgaccatgattacgcccaatttgcggccaagttcca

SEQ ID NO: 22 - DNA, 45 bp, Synthetic construct
  source 1..45: mol_type = other DNA
actagtcagatctaccattcaagaccttcttttttcaacttcgac

SEQ ID NO: 23 - DNA, 41 bp, Synthetic construct
  source 1..41: mol_type = other DNA
tatgaccatgattacgccgcttgtcttgcttgtttttgctc

SEQ ID NO: 24 - DNA, 46 bp, Synthetic construct
  source 1..46: mol_type = other DNA
actagtcagatctaccatttaagaccttcttttttcaacttcgaca

SEQ ID NO: 25 - DNA, 41 bp, Synthetic construct
  source 1..41: mol_type = other DNA
tatgaccatgattacgcccgataaggaaacgagagaggttg

SEQ ID NO: 26 - DNA, 42 bp, Synthetic construct
  source 1..42: mol_type = other DNA
actagtcagatctaccatgctgtaacgtttcagacaataacc

SEQ ID NO: 27 - DNA, 41 bp, Synthetic construct
  source 1..41: mol_type = other DNA
tatgaccatgattacgccgtgtgtttcggaaagcagcaaac

SEQ ID NO: 28 - DNA, 39 bp, Synthetic construct
  source 1..39: mol_type = other DNA
actagtcagatctaccatactgaaacccaggcatccacg

SEQ ID NO: 29 - DNA, 42 bp, Synthetic construct
  source 1..42: mol_type = other DNA
tatgaccatgattacgccgttaggtgacgactatatcagcat

SEQ ID NO: 30 - DNA, 43 bp, Synthetic construct
  source 1..43: mol_type = other DNA
actagtcagatctaccatgagagaaagatatcaaatcttgcac

SEQ ID NO: 31 - DNA, 42 bp, Synthetic construct
  source 1..42: mol_type = other DNA
tatgaccatgattacgccgctaatcttgaacaagtcctggat

SEQ ID NO: 32 - DNA, 42 bp, Synthetic construct
  source 1..42: mol_type = other DNA
actagtcagatctaccatggaagacgtgagatatgaatgcaa

SEQ ID NO: 33 - DNA, 42 bp, Synthetic construct
  source 1..42: mol_type = other DNA
tatgaccatgattacgccgtacctgtaattagtcaactgttc

SEQ ID NO: 34 - DNA, 40 bp, Synthetic construct
  source 1..40: mol_type = other DNA
actagtcagatctaccatcaccatctccaagatccaccac

SEQ ID NO: 35 - DNA, 19 bp, Synthetic construct
  source 1..19: mol_type = other DNA
gacgctggctcgcaacggt

SEQ ID NO: 36 - DNA, 20 bp, Synthetic construct
  source 1..20: mol_type = other DNA
cggccgccccaatccatacc

SEQ ID NO: 37 - DNA, 18 bp, Synthetic construct
  source 1..18: mol_type = other DNA
acgctgcctcgcaacggc

SEQ ID NO: 38 - DNA, 21 bp, Synthetic construct
  source 1..21: mol_type = other DNA
tggccgcccaagtccatacct

SEQ ID NO: 39 - DNA, 19 bp, Synthetic construct
  source 1..19: mol_type = other DNA
acgcctggctcgcaacggc

SEQ ID NO: 40 - DNA, 20 bp, Synthetic construct
  source 1..20: mol_type = other DNA
cggccgccccaatccatacc